European Patent Specification EP 3 795 180 B1, published November 5, 2025. Title: AAV-REP-1 FOR GENE THERAPY FOR CHOROIDEREMIA AND ACHROMATOPSIA. Applicant: Trustees of the University of Pennsylvania. Application PCT/US2016/066402. The sequence listing filed with the application follows.

SEQUENCE LISTING (29 sequences)

SEQ ID NO: 1 - DNA, 1962 bp, Artificial Sequence
  codon optimized sequence
  CDS (1)..(1962)
atggctgataccctgccctctgaattcgacgtgattgtgattggaaccggactccctgaatcgatcatcgccgcggcctgttcccggtccggtcggcgcgtgctgcacgtcgattcgagaagctactacggagggaattgggcctcattctccttctccggactgctctcctggctgaaggagtatcaggagaactccgacattgtctccgactcacctgtgtggcaggaccagatcctggaaaacgaggaagcaatagccctgagccggaaggacaagaccatccagcacgtggaggtgttctgttatgcctcccaagacctccatgaggacgtggaagaggctggagcgttgcagaagaatcatgccctcgtgacctccgctaactccaccgaggcagccgacagcgccttcctgccgaccgaggatgaatccctgtcaactatgtcgtgcgaaatgctgaccgaacagactccgagctccgaccccgaaaacgccctggaagtgaacggagcggaagtgaccggcgaaaaggagaaccattgcgacgacaagacttgtgtcccatccacttccgcggaggacatgtccgagaatgtgcctatcgccgaggacaccaccgaacagcccaagaagaacagaatcacgtacagccagatcatcaaggaggggcggaggtttaacatcgatctggtgtcgaagctgctgtacagccgcggtctgctgatcgatctgctcattaagtcgaacgtgtcgagatacgccgagttcaagaacatcacaaggattctcgccttccgggaaggaagagtggaacaagtgccgtgctcccgggccgacgtgttcaactcaaagcaacttaccatggtggaaaagcgcatgctgatgaaattcctgaccttctgcatggagtacgaaaagtaccctgatgagtacaagggttacgaagaaattactttctacgagtacctcaagacccagaagctgaccccgaatctgcagtacattgtgatgcactcaatcgcaatgacctccgaaaccgcctcctcgaccatcgacgggctcaaggccaccaagaacttcctgcactgtttggggcgctacggcaacactccgttcctcttcccgctgtacggccagggagagctgcctcagtgtttctgccggatgtgcgccgtgttcggcggaatctactgtctccgccactcggtccagtgcctggtggtggacaaggaatccaggaagtgcaaagccattattgaccagttcggacaacggatcatttccgagcactttcttgtggaggactcatacttcccggagaacatgtgctctcgggtccagtatcgacagatttccagggcggtgctcattactgaccggagcgtcctcaagaccgatagcgaccagcagatctccatcctgaccgtgccggcggaagaacccggcacttttgccgtgcgcgtgatcgagctttgctcatccaccatgacttgcatgaaaggcacttacctggtgcacctgacgtgcacctcatcgaaaaccgctagagaggacctggaatccgtcgtccaaaagctgttcgtgccttacaccgagatggaaattgaaaacgaacaagtggagaagccccgcatcctttgggccctgtactttaacatgcgcgattcctccgatatctcgcggtcctgctataacgacttgccttcgaacgtctacgtctgctccgggccagactgcggtcttggcaacgacaatgccgtgaagcaggcggaaacactgttccaagagatctgccctaacgaggatttttgcccgccccccccaaaccccgaggatatcatcttggacggagacagcctgcagccagaagcatccgagtccagcgccatcccggaggccaacagcgaaaccttcaaggagagcactaacctgggcaacctggaagagtccagcgaatga

SEQ ID NO: 2 - protein, 653 aa, Artificial Sequence
  Synthetic Construct
MADTLPSEFDVIVIGTGLPESIIAAACSRSGRRVLHVDSRSYYGGNWASFSFSGLLSWLKEYQENSDIVSDSPVWQDQILENEEAIALSRKDKTIQHVEVFCYASQDLHEDVEEAGALQKNHALVTSANSTEAADSAFLPTEDESLSTMSCEMLTEQTPSSDPENALEVNGAEVTGEKENHCDDKTCVPSTSAEDMSENVPIAEDTTEQPKKNRITYSQIIKEGRRFNIDLVSKLLYSRGLLIDLLIKSNVSRYAEFKNITRILAFREGRVEQVPCSRADVFNSKQLTMVEKRMLMKFLTFCMEYEKYPDEYKGYEEITFYEYLKTQKLTPNLQYIVMHSIAMTSETASSTIDGLKATKNFLHCLGRYGNTPFLFPLYGQGELPQCFCRMCAVFGGIYCLRHSVQCLVVDKESRKCKAIIDQFGQRIISEHFLVEDSYFPENMCSRVQYRQISRAVLITDRSVLKTDSDQQISILTVPAEEPGTFAVRVIELCSSTMTCMKGTYLVHLTCTSSKTAREDLESVVQKLFVPYTEMEIENEQVEKPRILWALYFNMRDSSDISRSCYNDLPSNVYVCSGPDCGLGNDNAVKQAETLFQEICPNEDFCPPPPNPEDIILDGDSLQPEASESSAIPEANSETFKESTNLGNLEESSE

SEQ ID NO: 3 - DNA, 1962 bp, Homo sapiens
  CDS (1)..(1962)
atggcggatactctcccttcggagtttgatgtgatcgtaatagggacgggtttgcctgaatccatcattgcagctgcatgttcaagaagtggccggagagttctgcatgttgattcaagaagctactatggaggaaactgggccagttttagcttttcaggactattgtcctggctaaaggaataccaggaaaacagtgacattgtaagtgacagtccagtgtggcaagaccagatccttgaaaatgaagaagccattgctcttagcaggaaggacaaaactattcaacatgtggaagtattttgttatgccagtcaggatttgcatgaagatgtcgaagaagctggtgcactgcagaaaaatcatgctcttgtgacatctgcaaactccacagaagctgcagattctgccttcctgcctacggaggatgagtcattaagcactatgagctgtgaaatgctcacagaacaaactccaagcagcgatccagagaatgcgctagaagtaaatggtgctgaagtgacaggggaaaaagaaaaccattgtgatgataaaacttgtgtgccatcaacttcagcagaagacatgagtgaaaatgtgcctatagcagaagataccacagagcaaccaaagaaaaacagaattacttactcacaaattattaaagaaggcaggagatttaatattgatttagtatcaaagctgctgtattctcgaggattactaattgatcttctaatcaaatctaatgttagtcgatatgcagagtttaaaaatattaccaggattcttgcatttcgagaaggacgagtggaacaggttccgtgttccagagcagatgtctttaatagcaaacaacttactatggtagaaaagcgaatgctaatgaaatttcttacattttgtatggaatatgagaaatatcctgatgaatataaaggatatgaagagatcacattttatgaatatttaaagactcaaaaattaacccccaacctccaatatattgtcatgcattcaattgcaatgacatcagagacagccagcagcaccatagatggtctcaaagctaccaaaaactttcttcactgtcttgggcggtatggcaacactccatttttgtttcctttatatggccaaggagaactcccccagtgtttctgcaggatgtgtgctgtgtttggtggaatttattgtcttcgccattcagtacagtgccttgtagtggacaaagaatccagaaaatgtaaagcaattatagatcagtttggtcagagaataatctctgagcatttcctcgtggaggacagttactttcctgagaacatgtgctcacgtgtgcaatacaggcagatctccagggcagtgctgattacagatagatctgtcctaaaaacagattcagatcaacagatttccattttgacagtgccagcagaggaaccaggaacttttgctgttcgggtcattgagttatgttcttcaacgatgacatgcatgaaaggcacctatttggttcatttgacttgcacatcttctaaaacagcaagagaagatttagaatcagttgtgcagaaattgtttgttccatatactgaaatggagatagaaaatgaacaagtagaaaagccaagaattctgtgggctctttacttcaatatgagagattcgtcagacatcagcaggagctgttataatgatttaccatccaacgtttatgtctgctctggcccagattgtggtttaggaaatgataatgcagtcaaacaggctgaaacacttttccaggaaatctgccccaatgaagatttctgtccccctccaccaaatcctgaagacattatccttgatggagacagtttacagccagaggcttcagaatccagtgccataccagaggctaactcggagactttcaaggaaagcacaaaccttggaaacctagaggagtcctctgaataa

SEQ ID NO: 4 - protein, 653 aa, Homo sapiens; identical to SEQ ID NO: 2

SEQ ID NO: 5 - DNA, 1985 bp, Artificial Sequence
  constructed plasmid
  misc_feature (1)..(8): NotI restriction site for subcloning into proviral plasmid
  misc_feature (4)..(16): Kozak consensus sequence
  CDS (13)..(1971): codon-optimized open reading frame (ORF)
  misc_feature (1972)..(1977): BclI restriction site with embedded stop codon/ site to add optional epitope tag
  misc_feature (1980)..(1985): BamHI restriction site for subcloning into proviral plasmid
gcggccgccaccatggctgataccctgccctctgaattcgacgtgattgtgattggaaccggactccctgaatcgatcatcgccgcggcctgttcccggtccggtcggcgcgtgctgcacgtcgattcgagaagctactacggagggaattgggcctcattctccttctccggactgctctcctggctgaaggagtatcaggagaactccgacattgtctccgactcacctgtgtggcaggaccagatcctggaaaacgaggaagcaatagccctgagccggaaggacaagaccatccagcacgtggaggtgttctgttatgcctcccaagacctccatgaggacgtggaagaggctggagcgttgcagaagaatcatgccctcgtgacctccgctaactccaccgaggcagccgacagcgccttcctgccgaccgaggatgaatccctgtcaactatgtcgtgcgaaatgctgaccgaacagactccgagctccgaccccgaaaacgccctggaagtgaacggagcggaagtgaccggcgaaaaggagaaccattgcgacgacaagacttgtgtcccatccacttccgcggaggacatgtccgagaatgtgcctatcgccgaggacaccaccgaacagcccaagaagaacagaatcacgtacagccagatcatcaaggaggggcggaggtttaacatcgatctggtgtcgaagctgctgtacagccgcggtctgctgatcgatctgctcattaagtcgaacgtgtcgagatacgccgagttcaagaacatcacaaggattctcgccttccgggaaggaagagtggaacaagtgccgtgctcccgggccgacgtgttcaactcaaagcaacttaccatggtggaaaagcgcatgctgatgaaattcctgaccttctgcatggagtacgaaaagtaccctgatgagtacaagggttacgaagaaattactttctacgagtacctcaagacccagaagctgaccccgaatctgcagtacattgtgatgcactcaatcgcaatgacctccgaaaccgcctcctcgaccatcgacgggctcaaggccaccaagaacttcctgcactgtttggggcgctacggcaacactccgttcctcttcccgctgtacggccagggagagctgcctcagtgtttctgccggatgtgcgccgtgttcggcggaatctactgtctccgccactcggtccagtgcctggtggtggacaaggaatccaggaagtgcaaagccattattgaccagttcggacaacggatcatttccgagcactttcttgtggaggactcatacttcccggagaacatgtgctctcgggtccagtatcgacagatttccagggcggtgctcattactgaccggagcgtcctcaagaccgatagcgaccagcagatctccatcctgaccgtgccggcggaagaacccggcacttttgccgtgcgcgtgatcgagctttgctcatccaccatgacttgcatgaaaggcacttacctggtgcacctgacgtgcacctcatcgaaaaccgctagagaggacctggaatccgtcgtccaaaagctgttcgtgccttacaccgagatggaaattgaaaacgaacaagtggagaagccccgcatcctttgggccctgtactttaacatgcgcgattcctccgatatctcgcggtcctgctataacgacttgccttcgaacgtctacgtctgctccgggccagactgcggtcttggcaacgacaatgccgtgaagcaggcggaaacactgttccaagagatctgccctaacgaggatttttgcccgccccccccaaaccccgaggatatcatcttggacggagacagcctgcagccagaagcatccgagtccagcgccatcccggaggccaacagcgaaaccttcaaggagagcactaacctgggcaacctggaagagtccagcgaatgatcataggatcc

SEQ ID NO: 6 - protein, 653 aa, Artificial Sequence; identical to SEQ ID NO: 2
  Synthetic Construct

SEQ ID NO: 7 - DNA, 9187 bp, Artificial Sequence
  constructed plasmid
  misc_feature (1)..(145): 5' ITR
  promoter (169)..(1786): CMV.CBA promoter
  misc_feature (1787)..(1794): Not I cloning site, cuts at 1789
  misc_feature (1805)..(1810): BamHI cloning site, cuts at 1806
  polyA_signal (1850)..(2052): BGH PolyA
  misc_feature (2109)..(2252): 3' ITR
  misc_feature (2571)..(6624): lambda stuffer
  misc_feature (7314)..(8126): Kanamycin resistance (complementary)
  misc_feature (8485)..(9128): Origin of replication (complementary)
tcgctcgctcactgaggccgcccgggcaaagcccgggcgtcgggcgacctttggtcgcccggcctcagtgagcgagcgagcgcgcagagagggagtggccaactccatcactaggggttcctgcggcctagtaggctcagaggcacacaggagtttctgcaaatctagtgcaggcgttacataacttacggtaaatggcccgcctggctgaccgcccaacgacccccgcccattgacgtcaataatgacgtatgttcccatagtaacgccaatagggactttccattgacgtcaatgggtggagtatttacggtaaactgcccacttggcagtacatcaagtgtatcatatgccaagtacgccccctattgacgtcaatgacggtaaatggcccgcctggcattatgcccagtacatgaccttatgggactttcctacttggcagtacatctacgtattagtcatcgctattaacatggtcgaggtgagccccacgttctgcttcactctccccatctcccccccctccccacccccaattttgtatttatttattttttaattattttgtgcagcgatgggggcggggggggggggggggcgcgcgccaggcggggcggggcggggcgaggggcggggcggggcgaggcggagaggtgcggcggcagccaatcagagcggcgcgctccgaaagtttccttttatggcgaggcggcggcggcggcggccctataaaaagcgaagcgcgcggcgggcggggagtcgctgcgacgctgccttcgccccgtgccccgctccgccgccgcctcgcgccgcccgccccggctctgactgaccgcgttactcccacaggtgagcgggcgggacggcccttctcctccgggctgtaattagcgcttggtttaatgacggcttgtttcttttctgtggctgcgtgaaagccttgaggggctccgggagggccctttgtgcggggggagcggctcggggggtgcgtgcgtgtgtgtgtgcgtggggagcgccgcgtgcggctccgcgctgcccggcggctgtgagcgctgcgggcgcggcgcggggctttgtgcgctccgcagtgtgcgcgaggggagcgcggccgggggcggtgccccgcggtgcggggggggctgcgaggggaacaaaggctgcgtgcggggtgtgtgcgtgggggggtgagcagggggtgtgggcgcgtcggtcgggctgcaaccccccctgcacccccctccccgagttgctgagcacggcccggcttcgggtgcggggctccgtacggggcgtggcgcggggctcgccgtgccgggcggggggtggcggcaggtgggggtgccgggcggggcggggccgcctcgggccggggagggctcgggggaggggcgcggcggcccccggagcgccggcggctgtcgaggcgcggcgagccgcagccattgccttttatggtaatcgtgcgagagggcgcagggacttcctttgtcccaaatctgtgcggagccgaaatctgggaggcgccgccgcaccccctctagcgggcgcggggcgaagcggtgcggcgccggcaggaaggaaatgggcggggagggccttcgtgcgtcgccgcgccgccgtccccttctccctctccagcctcggggctgtccgcggggggacggctgccttcgggggggacggggcagggcggggttcggcttctggcgtgtgaccggcggctctagacaattgtactaaccttcttctctttcctctcctgacaggttggtgtacactagcggccgcatagtactgcggatcctgcagatctcgagccgaattcctgcagcccgggggatcagcctcgactgtgccttctagttgccagccatctgttgtttgcccctcccccgtgccttccttgaccctggaaggtgccactcccactgtcctttcctaataaaatgaggaaattgcatcgcattgtctgagtaggtgtcattctattctggggggtggggtggggcaggacagcaagggggaggattgggaagacaatagcaggcatgctggggatgcggtgggctctatggcttctgaggcggaaagaaccagctggggctcgagatccactagggccgcaggaacccctagtgatggagttggccactccctctctgcgcgctcgctcgctcactgaggccgggcgaccaaaggtcgcccgacgcccgggctttgcccgggcggcctcagtgagcgagcgacctgcaggggcagcttgaaggaaatactaaggcaaaggtactgcaagtgctcgcaacattcgcttatgcggattattgccgtagtgccgcgacgccgggggcaagatgcagagattgccatggtacaggccgtgcggttgatattgccaaaacagagctgtgggggagagttgtcgagaaagagtgcggaagatgcaaaggcgtcggctattcaaggatgccagcaagcgcagcatatcgcgctgtgacgatgctaatcccaaaccttacccaacccacctggtcacgcactgttaagccgctgtatgacgctctggtggtgcaatgccacaaagaagagtcaatcgcagacaacattttgaatgcggtcacacgttagcagcatgattgccacggatggcaacatattaacggcatgatattgacttattgaataaaattgggtaaatttgactcaacgatgggttaattcgctcgttgtggtagtgagatgaaaagaggcggcgcttactaccgattccgcctagttggtcacttcgacgtatcgtctggaactccaaccatcgcaggcagagaggtctgcaaaatgcaatcccgaaacagttcgcaggtaatagttagagcctgcataacggtttcgggattttttatatctgcacaacaggtaagagcattgagtcgataatcgtgaagagtcggcgagcctggttagccagtgctctttccgttgtgctgaattaagcgaataccggaagcagaaccggatcaccaaatgcgtacaggcgtcatcgccgcccagcaacagcacaacccaaactgagccgtagccactgtctgtcctgaattcattagtaatagttacgctgcggccttttacacatgaccttcgtgaaagcgggtggcaggaggtcgcgctaacaacctcctgccgttttgcccgtgcatatcggtcacgaacaaatctgattactaaacacagtagcctggatttgttctatcagtaatcgaccttattcctaattaaatagagcaaatccccttattgggggtaagacatgaagatgccagaaaaacatgacctgttggccgccattctcgcggcaaaggaacaaggcatcggggcaatccttgcgtttgcaatggcgtaccttcgcggcagatataatggcggtgcgtttacaaaaacagtaatcgacgcaacgatgtgcgccattatcgcctggttcattcgtgaccttctcgacttcgccggactaagtagcaatctcgcttatataacgagcgtgtttatcggctacatcggtactgactcgattggttcgcttatcaaacgcttcgctgctaaaaaagccggagtagaagatggtagaaatcaataatcaacgtaaggcgttcctcgatatgctggcgtggtcggagggaactgataacggacgtcagaaaaccagaaatcatggttatgacgtcattgtaggcggagagctatttactgattactccgatcaccctcgcaaacttgtcacgctaaacccaaaactcaaatcaacaggcgccggacgctaccagcttctttcccgttggtgggatgcctaccgcaagcagcttggcctgaaagacttctctccgaaaagtcaggacgctgtggcattgcagcagattaaggagcgtggcgctttacctatgattgatcgtggtgatatccgtcaggcaatcgaccgttgcagcaatatctgggcttcactgccgggcgctggttatggtcagttcgagcataaggctgacagcctgattgcaaaattcaaagaagcgggcggaacggtcagagagattgatgtatgagcagagtcaccgcgattatctccgctctggttatctgcatcatcgtctgcctgtcatgggctgttaatcattaccgtgataacgccattacctacaaagcccagcgcgacaaaaatgccagagaactgaagctggcgaacgcggcaattactgacatgcagatgcgtcagcgtgatgttgctgcgctcgatgcaaaatacacgaaggagttagctgatgctaaagctgaaaatgatgctctgcgtgatgatgttgccgctggtcgtcgtcggttgcacatcaaagcagtctgtcagtcagtgcgtgaagccaccaccgcctccggcgtggataatgcagcctccccccgactggcagacaccgctgaacgggattatttcaccctcagagagaggctgatcactatgcaaaaacaactggaaggaacccagaagtatattaatgagcagtgcagatagagttgcccatatcgatgggcaactcatgcaattattgtgagcaatacacacgcgcttccagcggagtataaatgcctaaagtaataaaaccgagcaatccatttacgaatgtttgctgggtttctgttttaacaacattttctgcgccgccacaaattttggctgcatcgacagttttcttctgcccaattccagaaacgaagaaatgatgggtgatggtttcctttggtgctactgctgccggtttgttttgaacagtaaacgtctgttgagcacatcctgtaataagcagggccagcgcagtagcgagtagcatttttttcatggtgttattcccgatgctttttgaagttcgcagaatcgtatgtgtagaaaattaaacaaaccctaaacaatgagttgaaatttcatattgttaatatttattaatgtatgtcaggtgcgatgaatcgtcattgtattcccggattaactatgtccacagccctgacggggaacttctctgcgggagtgtccgggaataattaaaacgatgcacacagggtttagcgcgtacacgtattgcattatgccaacgccccggtgctgacacggaagaaaccggacgttatgatttagcgtggaaagatttgtgtagtgttctgaatgctctcagtaaatagtaatgaattatcaaaggtatagtaatatcttttatgttcatggatatttgtaacccatcggaaaactcctgctttagcaagattttccctgtattgctgaaatgtgatttctcttgatttcaacctatcataggacgtttctataagatgcgtgtttcttgagaatttaacatttacaacctttttaagtccttttattaacacggtgttatcgttttctaacacgatgtgaatattatctgtggctagatagtaaatataatgtgagacgttgtgacgttttagttcagaataaaacaattcacagtctaaatcttttcgcacttgatcgaatatttctttaaaaatggcaacctgagccattggtaaaaccttccatgtgatacgagggcgcgtagtttgcattatcgtttttatcgtttcaatctggtctgacctccttgtgttttgttgatgatttatgtcaaatattaggaatgttttcacttaatagtattggttgcgtaacaaagtgcggtcctgctggcattctggagggaaatacaaccgacagatgtatgtaaggccaacgtgctcaaatcttcatacagaaagatttgaagtaatattttaaccgctagatgaagagcaagcgcatggagcgacaaaatgaataaagaacaatctgctgatgatccctccgtggatctgattcgtgtaaaaaatatgcttaatagcaccatttctatgagttaccctgatgttgtaattgcatgtatagaacataaggtgtctctggaagcattcagagcaattgaggcagcgttggtgaagcacgataataatatgaaggattattccctggtggttgactgatcaccataactgctaatcattcaaactatttagtctgtgacagagccaacacgcagtctgtcactgtcaggaaagtggtaaaactgcaactcaattactgcaatgccctcgtaattaagtgaatttacaatatcgtcctgttcggagggaagaacgcgggatgttcattcttcatcacttttaattgatgtatatgctctcttttctgacgttagtctccgacggcaggcttcaatgacccaggctgagaaattcccggaccctttttgctcaagagcgatgttaatttgttcaatcatttggttaggaaagcggatgttgcgggttgttgttctgcgggttctgttcttcgttgacatgaggttgccccgtattcagtgtcgctgatttgtattgtctgaagttgtttttacgttaagttgatgcagatcaattaatacgatacctgcgtcataattgattatttgacgtggtttgatggcctccacgcacgttgtgatatgtagatgataatcattatcactttacgggtcctttccggtgatccgacaggttacggcctgatgcggtattttctccttacgcatctgtgcggtatttcacaccgcatacgtcaaagcaaccatagtacgcgccctgtagcggcgcattaagcgcggcgggtgtggtggttacgcgcagcgtgaccgctacacttgccagcgccctagcgcccgctcctttcgctttcttcccttcctttctcgccacgttcgccggctttccccgtcaagctctaaatcgggggctccctttagggttccgatttagtgctttacggcacctcgaccccaaaaaacttgatttgggtgatggttcacgtagtgggccatcgccctgatagacggtttttcgccctttgacgttggagtccacgttctttaatagtggactcttgttccaaactggaacaacactcaaccctatctcgggctattcttttgatttagacctgcaggcatgcaagcttactggccgtcgttttacaacgtcgtgactgggaaaaccctggcgttacccaacttaatcgccttgcagcacatccccctttcgccagctggcgtaatagcgaagaggcccgcaccgatcgcccttcccaacagttgcgcagcctgaatggcgaatgcgatttattcaacaaagccgccgtcccgtcaagtcagcgtaatgctctgccagtgttacaaccaattaaccaattctgattagaaaaactcatcgagcatcaaatgaaactgcaatttattcatatcaggattatcaataccatatttttgaaaaagccgtttctgtaatgaaggagaaaactcaccgaggcagttccataggatggcaagatcctggtatcggtctgcgattccgactcgtccaacatcaatacaacctattaatttcccctcgtcaaaaataaggttatcaagtgagaaatcaccatgagtgacgactgaatccggtgagaatggcaaaagcttatgcatttctttccagacttgttcaacaggccagccattacgctcgtcatcaaaatcactcgcatcaaccaaaccgttattcattcgtgattgcgcctgagcgagacgaaatacgcgatcgctgttaaaaggacaattacaaacaggaatcgaatgcaaccggcgcaggaacactgccagcgcatcaacaatattttcacctgaatcaggatattcttctaatacctggaatgctgttttcccggggatcgcagtggtgagtaaccatgcatcatcaggagtacggataaaatgcttgatggtcggaagaggcataaattccgtcagccagtttagtctgaccatctcatctgtaacatcattggcaacgctacctttgccatgtttcagaaacaactctggcgcatcgggcttcccatacaatcgatagattgtcgcacctgattgcccgacattatcgcgagcccatttatacccatataaatcagcatccatgttggaatttaatcgcggcttcgagcaagacgtttcccgttgaatatggctcataacaccccttgtattactgtttatgtaagcagacagttttattgttcatgatgatatatttttatcttgtgcaatgtaacatcagagattttgagacacaacgtggctttgttgaataaatcgaacttttgctgagttgaaggatcagatcacgcatcttcccgacaacgcagaccgttccgtggcaaagcaaaagttcaaaatcaccaactggtccacctacaacaaagctctcatcaaccgtggctccctcactttctggctggatgatggggcgattcaggcctggtatgagtcagcaacaccttcttcacgaggcagacctctcgacggatcgttccactgagcgtcagaccccgtagaaaagatcaaaggatcttcttgagatcctttttttctgcgcgtaatctgctgcttgcaaacaaaaaaaccaccgctaccagcggtggtttgtttgccggatcaagagctaccaactctttttccgaaggtaactggcttcagcagagcgcagataccaaatactgtccttctagtgtagccgtagttaggccaccacttcaagaactctgtagcaccgcctacatacctcgctctgctaatcctgttaccagtggctgctgccagtggcgataagtcgtgtcttaccgggttggactcaagacgatagttaccggataaggcgcagcggtcgggctgaacggggggttcgtgcacacagcccagcttggagcgaacgacctacaccgaactgagatacctacagcgtgagctatgagaaagcgccacgcttcccgaagggagaaaggcggacaggtatccggtaagcggcagggtcggaacaggagagcgcacgagggagcttccagggggaaacgcctggtatctttatagtcctgtcgggtttcgccacctctgacttgagcgtcgatttttgtgatgctcgtcaggggggcggagcctatggaaaaacgccagcaacgcggcctttttacggttcctggccttttgctggccttttgctcacatgtcctgcaggcagctgcgcgccagctgcgcgc

SEQ ID NO: 8 - DNA, 11148 bp, Artificial Sequence
  constructed plasmid
tcgctcgctcactgaggccgcccgggcaaagcccgggcgtcgggcgacctttggtcgcccggcctcagtgagcgagcgagcgcgcagagagggagtggccaactccatcactaggggttcctgcggcctagtaggctcagaggcacacaggagtttctgcaaatctagtgcaggcgttacataacttacggtaaatggcccgcctggctgaccgcccaacgacccccgcccattgacgtcaataatgacgtatgttcccatagtaacgccaatagggactttccattgacgtcaatgggtggagtatttacggtaaactgcccacttggcagtacatcaagtgtatcatatgccaagtacgccccctattgacgtcaatgacggtaaatggcccgcctggcattatgcccagtacatgaccttatgggactttcctacttggcagtacatctacgtattagtcatcgctattaacatggtcgaggtgagccccacgttctgcttcactctccccatctcccccccctccccacccccaattttgtatttatttattttttaattattttgtgcagcgatgggggcggggggggggggggggcgcgcgccaggcggggcggggcggggcgaggggcggggcggggcgaggcggagaggtgcggcggcagccaatcagagcggcgcgctccgaaagtttccttttatggcgaggcggcggcggcggcggccctataaaaagcgaagcgcgcggcgggcggggagtcgctgcgacgctgccttcgccccgtgccccgctccgccgccgcctcgcgccgcccgccccggctctgactgaccgcgttactcccacaggtgagcgggcgggacggcccttctcctccgggctgtaattagcgcttggtttaatgacggcttgtttcttttctgtggctgcgtgaaagccttgaggggctccgggagggccctttgtgcggggggagcggctcggggggtgcgtgcgtgtgtgtgtgcgtggggagcgccgcgtgcggctccgcgctgcccggcggctgtgagcgctgcgggcgcggcgcggggctttgtgcgctccgcagtgtgcgcgaggggagcgcggccgggggcggtgccccgcggtgcggggggggctgcgaggggaacaaaggctgcgtgcggggtgtgtgcgtgggggggtgagcagggggtgtgggcgcgtcggtcgggctgcaaccccccctgcacccccctccccgagttgctgagcacggcccggcttcgggtgcggggctccgtacggggcgtggcgcggggctcgccgtgccgggcggggggtggcggcaggtgggggtgccgggcggggcggggccgcctcgggccggggagggctcgggggaggggcgcggcggcccccggagcgccggcggctgtcgaggcgcggcgagccgcagccattgccttttatggtaatcgtgcgagagggcgcagggacttcctttgtcccaaatctgtgcggagccgaaatctgggaggcgccgccgcaccccctctagcgggcgcggggcgaagcggtgcggcgccggcaggaaggaaatgggcggggagggccttcgtgcgtcgccgcgccgccgtccccttctccctctccagcctcggggctgtccgcggggggacggctgccttcgggggggacggggcagggcggggttcggcttctggcgtgtgaccggcggctctagacaattgtactaaccttcttctctttcctctcctgacaggttggtgtacactagcggccgccaccatggctgataccctgccctctgaattcgacgtgattgtgattggaaccggactccctgaatcgatcatcgccgcggcctgttcccggtccggtcggcgcgtgctgcacgtcgattcgagaagctactacggagggaattgggcctcattctccttctccggactgctctcctggctgaaggagtatcaggagaactccgacattgtctccgactcacctgtgtggcaggaccagatcctggaaaacgaggaagcaatagccctgagccggaaggacaagaccatccagcacgtggaggtgttctgttatgcctcccaagacctccatgaggacgtggaagaggctggagcgttgcagaagaatcatgccctcgtgacctccgctaactccaccgaggcagccgacagcgccttcctgccgaccgaggatgaatccctgtcaactatgtcgtgcgaaatgctgaccgaacagactccgagctccgaccccgaaaacgccctggaagtgaacggagcggaagtgaccggcgaaaaggagaaccattgcgacgacaagacttgtgtcccatccacttccgcggaggacatgtccgagaatgtgcctatcgccgaggacaccaccgaacagcccaagaagaacagaatcacgtacagccagatcatcaaggaggggcggaggtttaacatcgatctggtgtcgaagctgctgtacagccgcggtctgctgatcgatctgctcattaagtcgaacgtgtcgagatacgccgagttcaagaacatcacaaggattctcgccttccgggaaggaagagtggaacaagtgccgtgctcccgggccgacgtgttcaactcaaagcaacttaccatggtggaaaagcgcatgctgatgaaattcctgaccttctgcatggagtacgaaaagtaccctgatgagtacaagggttacgaagaaattactttctacgagtacctcaagacccagaagctgaccccgaatctgcagtacattgtgatgcactcaatcgcaatgacctccgaaaccgcctcctcgaccatcgacgggctcaaggccaccaagaacttcctgcactgtttggggcgctacggcaacactccgttcctcttcccgctgtacggccagggagagctgcctcagtgtttctgccggatgtgcgccgtgttcggcggaatctactgtctccgccactcggtccagtgcctggtggtggacaaggaatccaggaagtgcaaagccattattgaccagttcggacaacggatcatttccgagcactttcttgtggaggactcatacttcccggagaacatgtgctctcgggtccagtatcgacagatttccagggcggtgctcattactgaccggagcgtcctcaagaccgatagcgaccagcagatctccatcctgaccgtgccggcggaagaacccggcacttttgccgtgcgcgtgatcgagctttgctcatccaccatgacttgcatgaaaggcacttacctggtgcacctgacgtgcacctcatcgaaaaccgctagagaggacctggaatccgtcgtccaaaagctgttcgtgccttacaccgagatggaaattgaaaacgaacaagtggagaagccccgcatcctttgggccctgtactttaacatgcgcgattcctccgatatctcgcggtcctgctataacgacttgccttcgaacgtctacgtctgctccgggccagactgcggtcttggcaacgacaatgccgtgaagcaggcggaaacactgttccaagagatctgccctaacgaggatttttgcccgccccccccaaaccccgaggatatcatcttggacggagacagcctgcagccagaagcatccgagtccagcgccatcccggaggccaacagcgaaaccttcaaggagagcactaacctgggcaacctggaagagtccagcgaatgatcataggatcctgcagatctcgagccgaattcctgcagcccgggggatcagcctcgactgtgccttctagttgccagccatctgttgtttgcccctcccccgtgccttccttgaccctggaaggtgccactcccactgtcctttcctaataaaatgaggaaattgcatcgcattgtctgagtaggtgtcattctattctggggggtggggtggggcaggacagcaagggggaggattgggaagacaatagcaggcatgctggggatgcggtgggctctatggcttctgaggcggaaagaaccagctggggctcgagatccactagggccgcaggaacccctagtgatggagttggccactccctctctgcgcgctcgctcgctcactgaggccgggcgaccaaaggtcgcccgacgcccgggctttgcccgggcggcctcagtgagcgagcgacctgcaggggcagcttgaaggaaatactaaggcaaaggtactgcaagtgctcgcaacattcgcttatgcggattattgccgtagtgccgcgacgccgggggcaagatgcagagattgccatggtacaggccgtgcggttgatattgccaaaacagagctgtgggggagagttgtcgagaaagagtgcggaagatgcaaaggcgtcggctattcaaggatgccagcaagcgcagcatatcgcgctgtgacgatgctaatcccaaaccttacccaacccacctggtcacgcactgttaagccgctgtatgacgctctggtggtgcaatgccacaaagaagagtcaatcgcagacaacattttgaatgcggtcacacgttagcagcatgattgccacggatggcaacatattaacggcatgatattgacttattgaataaaattgggtaaatttgactcaacgatgggttaattcgctcgttgtggtagtgagatgaaaagaggcggcgcttactaccgattccgcctagttggtcacttcgacgtatcgtctggaactccaaccatcgcaggcagagaggtctgcaaaatgcaatcccgaaacagttcgcaggtaatagttagagcctgcataacggtttcgggattttttatatctgcacaacaggtaagagcattgagtcgataatcgtgaagagtcggcgagcctggttagccagtgctctttccgttgtgctgaattaagcgaataccggaagcagaaccggatcaccaaatgcgtacaggcgtcatcgccgcccagcaacagcacaacccaaactgagccgtagccactgtctgtcctgaattcattagtaatagttacgctgcggccttttacacatgaccttcgtgaaagcgggtggcaggaggtcgcgctaacaacctcctgccgttttgcccgtgcatatcggtcacgaacaaatctgattactaaacacagtagcctggatttgttctatcagtaatcgaccttattcctaattaaatagagcaaatccccttattgggggtaagacatgaagatgccagaaaaacatgacctgttggccgccattctcgcggcaaaggaacaaggcatcggggcaatccttgcgtttgcaatggcgtaccttcgcggcagatataatggcggtgcgtttacaaaaacagtaatcgacgcaacgatgtgcgccattatcgcctggttcattcgtgaccttctcgacttcgccggactaagtagcaatctcgcttatataacgagcgtgtttatcggctacatcggtactgactcgattggttcgcttatcaaacgcttcgctgctaaaaaagccggagtagaagatggtagaaatcaataatcaacgtaaggcgttcctcgatatgctggcgtggtcggagggaactgataacggacgtcagaaaaccagaaatcatggttatgacgtcattgtaggcggagagctatttactgattactccgatcaccctcgcaaacttgtcacgctaaacccaaaactcaaatcaacaggcgccggacgctaccagcttctttcccgttggtgggatgcctaccgcaagcagcttggcctgaaagacttctctccgaaaagtcaggacgctgtggcattgcagcagattaaggagcgtggcgctttacctatgattgatcgtggtgatatccgtcaggcaatcgaccgttgcagcaatatctgggcttcactgccgggcgctggttatggtcagttcgagcataaggctgacagcctgattgcaaaattcaaagaagcgggcggaacggtcagagagattgatgtatgagcagagtcaccgcgattatctccgctctggttatctgcatcatcgtctgcctgtcatgggctgttaatcattaccgtgataacgccattacctacaaagcccagcgcgacaaaaatgccagagaactgaagctggcgaacgcggcaattactgacatgcagatgcgtcagcgtgatgttgctgcgctcgatgcaaaatacacgaaggagttagctgatgctaaagctgaaaatgatgctctgcgtgatgatgttgccgctggtcgtcgtcggttgcacatcaaagcagtctgtcagtcagtgcgtgaagccaccaccgcctccggcgtggataatgcagcctccccccgactggcagacaccgctgaacgggattatttcaccctcagagagaggctgatcactatgcaaaaacaactggaaggaacccagaagtatattaatgagcagtgcagatagagttgcccatatcgatgggcaactcatgcaattattgtgagcaatacacacgcgcttccagcggagtataaatgcctaaagtaataaaaccgagcaatccatttacgaatgtttgctgggtttctgttttaacaacattttctgcgccgccacaaattttggctgcatcgacagttttcttctgcccaattccagaaacgaagaaatgatgggtgatggtttcctttggtgctactgctgccggtttgttttgaacagtaaacgtctgttgagcacatcctgtaataagcagggccagcgcagtagcgagtagcatttttttcatggtgttattcccgatgctttttgaagttcgcagaatcgtatgtgtagaaaattaaacaaaccctaaacaatgagttgaaatttcatattgttaatatttattaatgtatgtcaggtgcgatgaatcgtcattgtattcccggattaactatgtccacagccctgacggggaacttctctgcgggagtgtccgggaataattaaaacgatgcacacagggtttagcgcgtacacgtattgcattatgccaacgccccggtgctgacacggaagaaaccggacgttatgatttagcgtggaaagatttgtgtagtgttctgaatgctctcagtaaatagtaatgaattatcaaaggtatagtaatatcttttatgttcatggatatttgtaacccatcggaaaactcctgctttagcaagattttccctgtattgctgaaatgtgatttctcttgatttcaacctatcataggacgtttctataagatgcgtgtttcttgagaatttaacatttacaacctttttaagtccttttattaacacggtgttatcgttttctaacacgatgtgaatattatctgtggctagatagtaaatataatgtgagacgttgtgacgttttagttcagaataaaacaattcacagtctaaatcttttcgcacttgatcgaatatttctttaaaaatggcaacctgagccattggtaaaaccttccatgtgatacgagggcgcgtagtttgcattatcgtttttatcgtttcaatctggtctgacctccttgtgttttgttgatgatttatgtcaaatattaggaatgttttcacttaatagtattggttgcgtaacaaagtgcggtcctgctggcattctggagggaaatacaaccgacagatgtatgtaaggccaacgtgctcaaatcttcatacagaaagatttgaagtaatattttaaccgctagatgaagagcaagcgcatggagcgacaaaatgaataaagaacaatctgctgatgatccctccgtggatctgattcgtgtaaaaaatatgcttaatagcaccatttctatgagttaccctgatgttgtaattgcatgtatagaacataaggtgtctctggaagcattcagagcaattgaggcagcgttggtgaagcacgataataatatgaaggattattccctggtggttgactgatcaccataactgctaatcattcaaactatttagtctgtgacagagccaacacgcagtctgtcactgtcaggaaagtggtaaaactgcaactcaattactgcaatgccctcgtaattaagtgaatttacaatatcgtcctgttcggagggaagaacgcgggatgttcattcttcatcacttttaattgatgtatatgctctcttttctgacgttagtctccgacggcaggcttcaatgacccaggctgagaaattcccggaccctttttgctcaagagcgatgttaatttgttcaatcatttggttaggaaagcggatgttgcgggttgttgttctgcgggttctgttcttcgttgacatgaggttgccccgtattcagtgtcgctgatttgtattgtctgaagttgtttttacgttaagttgatgcagatcaattaatacgatacctgcgtcataattgattatttgacgtggtttgatggcctccacgcacgttgtgatatgtagatgataatcattatcactttacgggtcctttccggtgatccgacaggttacggcctgatgcggtattttctccttacgcatctgtgcggtatttcacaccgcatacgtcaaagcaaccatagtacgcgccctgtagcggcgcattaagcgcggcgggtgtggtggttacgcgcagcgtgaccgctacacttgccagcgccctagcgcccgctcctttcgctttcttcccttcctttctcgccacgttcgccggctttccccgtcaagctctaaatcgggggctccctttagggttccgatttagtgctttacggcacctcgaccccaaaaaacttgatttgggtgatggttcacgtagtgggccatcgccctgatagacggtttttcgccctttgacgttggagtccacgttctttaatagtggactcttgttccaaactggaacaacactcaaccctatctcgggctattcttttgatttagacctgcaggcatgcaagcttactggccgtcgttttacaacgtcgtgactgggaaaaccctggcgttacccaacttaatcgccttgcagcacatccccctttcgccagctggcgtaatagcgaagaggcccgcaccgatcgcccttcccaacagttgcgcagcctgaatggcgaatgcgatttattcaacaaagccgccgtcccgtcaagtcagcgtaatgctctgccagtgttacaaccaattaaccaattctgattagaaaaactcatcgagcatcaaatgaaactgcaatttattcatatcaggattatcaataccatatttttgaaaaagccgtttctgtaatgaaggagaaaactcaccgaggcagttccataggatggcaagatcctggtatcggtctgcgattccgactcgtccaacatcaatacaacctattaatttcccctcgtcaaaaataaggttatcaagtgagaaatcaccatgagtgacgactgaatccggtgagaatggcaaaagcttatgcatttctttccagacttgttcaacaggccagccattacgctcgtcatcaaaatcactcgcatcaaccaaaccgttattcattcgtgattgcgcctgagcgagacgaaatacgcgatcgctgttaaaaggacaattacaaacaggaatcgaatgcaaccggcgcaggaacactgccagcgcatcaacaatattttcacctgaatcaggatattcttctaatacctggaatgctgttttcccggggatcgcagtggtgagtaaccatgcatcatcaggagtacggataaaatgcttgatggtcggaagaggcataaattccgtcagccagtttagtctgaccatctcatctgtaacatcattggcaacgctacctttgccatgtttcagaaacaactctggcgcatcgggcttcccatacaatcgatagattgtcgcacctgattgcccgacattatcgcgagcccatttatacccatataaatcagcatccatgttggaatttaatcgcggcttcgagcaagacgtttcccgttgaatatggctcataacaccccttgtattactgtttatgtaagcagacagttttattgttcatgatgatatatttttatcttgtgcaatgtaacatcagagattttgagacacaacgtggctttgttgaataaatcgaacttttgctgagttgaaggatcagatcacgcatcttcccgacaacgcagaccgttccgtggcaaagcaaaagttcaaaatcaccaactggtccacctacaacaaagctctcatcaaccgtggctccctcactttctggctggatgatggggcgattcaggcctggtatgagtcagcaacaccttcttcacgaggcagacctctcgacggatcgttccactgagcgtcagaccccgtagaaaagatcaaaggatcttcttgagatcctttttttctgcgcgtaatctgctgcttgcaaacaaaaaaaccaccgctaccagcggtggtttgtttgccggatcaagagctaccaactctttttccgaaggtaactggcttcagcagagcgcagataccaaatactgtccttctagtgtagccgtagttaggccaccacttcaagaactctgtagcaccgcctacatacctcgctctgctaatcctgttaccagtggctgctgccagtggcgataagtcgtgtcttaccgggttggactcaagacgatagttaccggataaggcgcagcggtcgggctgaacggggggttcgtgcacacagcccagcttggagcgaacgacctacaccgaactgagatacctacagcgtgagctatgagaaagcgccacgcttcccgaagggagaaaggcggacaggtatccggtaagcggcagggtcggaacaggagagcgcacgagggagcttccagggggaaacgcctggtatctttatagtcctgtcgggtttcgccacctctgacttgagcgtcgatttttgtgatgctcgtcaggggggcggagcctatggaaaaacgccagcaacgcggcctttttacggttcctggccttttgctggccttttgctcacatgtcctgcaggcagctgcgcgccagctgcgcgc

SEQ ID NO: 9 - DNA, 2085 bp, Artificial Sequence
  codon optimized sequence
  CDS (1)..(2085): codon-optimized ORF
atggctaagattaacacccagtactcacatccatcccgcactcacctcaaagtcaagacctccgatcgggatctgaaccgggctgagaatgggctgtcgcgcgcccactcgtcgtccgaggaaaccagcagcgtgctccagccgggcatcgccatggaaactagggggctggcggactccggacagggatccttcactggacagggtattgcccggctgagcagactgatcttcctgcttcgccgctgggcggccagacacgtgcaccatcaggaccagggacctgatagcttccccgaccgctttaggggagccgagctgaaagaagtgtcaagccaggagtcaaacgcgcaggccaacgtcggcagccaagagcctgcagaccggggacgctcggcatggccgctcgcaaagtgcaacactaacacttccaacaacaccgaagaggaaaagaaaaccaagaagaaggatgcaattgtggtggacccttcctccaacctgtactaccgctggttgaccgccatcgccctcccggtcttttacaattggtatctccttatctgccgggcctgcttcgacgaactgcaatcagagtacctgatgctgtggctggtgctggactatagcgccgatgtgctctacgtcctggatgtgctcgtgcgcgcccggaccggattcttggaacaaggcctgatggtgtccgacacgaatagactgtggcagcactataagaccacaacccagttcaagcttgacgtgctcagccttgtgccgactgacctggcctacctgaaagtcggaactaactacccggaagtcagattcaaccgactcctgaagttcagcaggctgttcgagttctttgaccgcaccgagactcggaccaactaccctaacatgttccggatcggaaatctggtgctctacatactgattatcatccattggaacgcctgtatctatttcgccatttcgaagttcatcggtttcggaaccgattcctgggtgtaccccaacatctcgatccccgaacacggtcgcctgtcccggaagtacatctactccctgtactggtccactctgactctgaccacgatcggggaaacccctccacccgtgaaggacgaagagtacctgttcgtggtggtggacttcctggtcggagtgttgattttcgccaccattgtgggaaacgtgggctccatgatctccaacatgaacgcgtcgagagctgagttccaagccaagatcgactccattaagcagtacatgcagttcagaaaggtcaccaaggacctggaaaccagggtcatccgctggttcgactacctgtgggccaacaaaaagactgtggacgaaaaggaagtgctgaagtcgctgccggataagctgaaggccgaaatcgccattaacgtgcaccttgacaccctgaagaaagtccggatcttccaagactgtgaagccggcctcctggtggagctcgtgctcaagctgcggcccaccgtgttcagcccgggagattacatttgcaagaagggcgatatcggcaaagagatgtacatcatcaacgagggaaagctggccgtggtcgcggacgacggcgtgacccagttcgtggtgctgtccgacggatcctacttcggtgaaatctcaatcctcaacatcaaggggtccaagtccggcaaccggagaactgccaacattcgctccatcggatacagcgacctgttttgcctgtccaaggatgacctgatggaggctctgactgagtaccctgaagcgaagaaggctttggaggaaaaggggcggcagattctgatgaaggacaatttgatcgacgaggagctcgcacgggccggcgccgaccccaaggatctcgaagagaaggtcgaacagctgggttcttcgcttgataccctgcaaacccgattcgcgcggctgctcgccgagtacaacgcgacccagatgaagatgaagcagagactgtcacagttggaatcccaagtcaagggcggaggcgacaagccgctggcggacggggaagtgcccggggacgccaccaagactgaggacaagcagcagtga

SEQ ID NO: 10 - protein, 694 aa, Artificial Sequence
  Synthetic Construct
MAKINTQYSHPSRTHLKVKTSDRDLNRAENGLSRAHSSSEETSSVLQPGIAMETRGLADSGQGSFTGQGIARLSRLIFLLRRWAARHVHHQDQGPDSFPDRFRGAELKEVSSQESNAQANVGSQEPADRGRSAWPLAKCNTNTSNNTEEEKKTKKKDAIVVDPSSNLYYRWLTAIALPVFYNWYLLICRACFDELQSEYLMLWLVLDYSADVLYVLDVLVRARTGFLEQGLMVSDTNRLWQHYKTTTQFKLDVLSLVPTDLAYLKVGTNYPEVRFNRLLKFSRLFEFFDRTETRTNYPNMFRIGNLVLYILIIIHWNACIYFAISKFIGFGTDSWVYPNISIPEHGRLSRKYIYSLYWSTLTLTTIGETPPPVKDEEYLFVVVDFLVGVLIFATIVGNVGSMISNMNASRAEFQAKIDSIKQYMQFRKVTKDLETRVIRWFDYLWANKKTVDEKEVLKSLPDKLKAEIAINVHLDTLKKVRIFQDCEAGLLVELVLKLRPTVFSPGDYICKKGDIGKEMYIINEGKLAVVADDGVTQFVVLSDGSYFGEISILNIKGSKSGNRRTANIRSIGYSDLFCLSKDDLMEALTEYPEAKKALEEKGRQILMKDNLIDEELARAGADPKDLEEKVEQLGSSLDTLQTRFARLLAEYNATQMKMKQRLSQLESQVKGGGDKPLADGEVPGDATKTEDKQQ

SEQ ID NO: 11 - DNA, 2250 bp, Artificial Sequence
  codon optimized sequence
  CDS (1)..(2250): codon-optimized ORF
atggctaagattaacacccagtactcacatccatcccgcactcacctcaaagtcaagacctccgatcgggatctgaaccgggctgagaatgggctgtcgcgcgcccactcgtcgtccgaggaaaccagcagcgtgctccagccgggcatcgccatggaaactagggggctggcggactccggacagggatccttcactggacagggtattgcccggttcgggcggattcagaagaagtcccagccggagaaggtcgtgcgggctgccagcaggggcaggccactcattggttggacacagtggtgcgctgaggatggtggagatgaatcggaaatggcactggccggctctcccggatgcagctcgggcccccaagggagactgagcagactgatcttcctgcttcgccgctgggcggccagacacgtgcaccatcaggaccagggacctgatagcttccccgaccgctttaggggagccgagctgaaagaagtgtcaagccaggagtcaaacgcgcaggccaacgtcggcagccaagagcctgcagaccggggacgctcggcatggccgctcgcaaagtgcaacactaacacttccaacaacaccgaagaggaaaagaaaaccaagaagaaggatgcaattgtggtggacccttcctccaacctgtactaccgctggttgaccgccatcgccctcccggtcttttacaattggtatctccttatctgccgggcctgcttcgacgaactgcaatcagagtacctgatgctgtggctggtgctggactatagcgccgatgtgctctacgtcctggatgtgctcgtgcgcgcccggaccggattcttggaacaaggcctgatggtgtccgacacgaatagactgtggcagcactataagaccacaacccagttcaagcttgacgtgctcagccttgtgccgactgacctggcctacctgaaagtcggaactaactacccggaagtcagattcaaccgactcctgaagttcagcaggctgttcgagttctttgaccgcaccgagactcggaccaactaccctaacatgttccggatcggaaatctggtgctctacatactgattatcatccattggaacgcctgtatctatttcgccatttcgaagttcatcggtttcggaaccgattcctgggtgtaccccaacatctcgatccccgaacacggtcgcctgtcccggaagtacatctactccctgtactggtccactctgactctgaccacgatcggggaaacccctccacccgtgaaggacgaagagtacctgttcgtggtggtggacttcctggtcggagtgttgattttcgccaccattgtgggaaacgtgggctccatgatctccaacatgaacgcgtcgagagctgagttccaagccaagatcgactccattaagcagtacatgcagttcagaaaggtcaccaaggacctggaaaccagggtcatccgctggttcgactacctgtgggccaacaaaaagactgtggacgaaaaggaagtgctgaagtcgctgccggataagctgaaggccgaaatcgccattaacgtgcaccttgacaccctgaagaaagtccggatcttccaagactgtgaagccggcctcctggtggagctcgtgctcaagctgcggcccaccgtgttcagcccgggagattacatttgcaagaagggcgatatcggcaaagagatgtacatcatcaacgagggaaagctggccgtggtcgcggacgacggcgtgacccagttcgtggtgctgtccgacggatcctacttcggtgaaatctcaatcctcaacatcaaggggtccaagtccggcaaccggagaactgccaacattcgctccatcggatacagcgacctgttttgcctgtccaaggatgacctgatggaggctctgactgagtaccctgaagcgaagaaggctttggaggaaaaggggcggcagattctgatgaaggacaatttgatcgacgaggagctcgcacgggccggcgccgaccccaaggatctcgaagagaaggtcgaacagctgggttcttcgcttgataccctgcaaacccgattcgcgcggctgctcgccgagtacaacgcgacccagatgaagatgaagcagagactgtcacagttggaatcccaagtcaagggcggaggcgacaagccgctggcggacggggaagtgcccggggacgccaccaagactgaggacaagcagcagtga

SEQ ID NO: 12 - protein, 749 aa, Artificial Sequence
  Synthetic Construct
MAKINTQYSHPSRTHLKVKTSDRDLNRAENGLSRAHSSSEETSSVLQPGIAMETRGLADSGQGSFTGQGIARFGRIQKKSQPEKVVRAASRGRPLIGWTQWCAEDGGDESEMALAGSPGCSSGPQGRLSRLIFLLRRWAARHVHHQDQGPDSFPDRFRGAELKEVSSQESNAQANVGSQEPADRGRSAWPLAKCNTNTSNNTEEEKKTKKKDAIVVDPSSNLYYRWLTAIALPVFYNWYLLICRACFDELQSEYLMLWLVLDYSADVLYVLDVLVRARTGFLEQGLMVSDTNRLWQHYKTTTQFKLDVLSLVPTDLAYLKVGTNYPEVRFNRLLKFSRLFEFFDRTETRTNYPNMFRIGNLVLYILIIIHWNACIYFAISKFIGFGTDSWVYPNISIPEHGRLSRKYIYSLYWSTLTLTTIGETPPPVKDEEYLFVVVDFLVGVLIFATIVGNVGSMISNMNASRAEFQAKIDSIKQYMQFRKVTKDLETRVIRWFDYLWANKKTVDEKEVLKSLPDKLKAEIAINVHLDTLKKVRIFQDCEAGLLVELVLKLRPTVFSPGDYICKKGDIGKEMYIINEGKLAVVADDGVTQFVVLSDGSYFGEISILNIKGSKSGNRRTANIRSIGYSDLFCLSKDDLMEALTEYPEAKKALEEKGRQILMKDNLIDEELARAGADPKDLEEKVEQLGSSLDTLQTRFARLLAEYNATQMKMKQRLSQLESQVKGGGDKPLADGEVPGDATKTEDKQQ

SEQ ID NO: 13 - DNA, 2085 bp, Homo sapiens
  CDS (1)..(2085): native open reading frame (ORF)
atggccaagatcaacacccaatactcccacccctccaggacccacctcaaggtaaagacctcagaccgggatctcaatcgcgctgaaaatggcctcagcagagcccactcgtcaagtgaggagacatcgtcagtgctgcagccggggatcgccatggagaccagaggactggctgactccgggcagggctccttcaccggccaggggatcgccaggctgtcgcgcctcatcttcttgctgcgcaggtgggctgccaggcatgtgcaccaccaggaccagggaccggactcttttcctgatcgtttccgtggagccgagcttaaggaggtgtccagccaagaaagcaatgcccaggcaaatgtgggcagccaggagccagcagacagagggagaagcgcctggcccctggccaaatgcaacactaacaccagcaacaacacggaggaggagaagaagacgaaaaagaaggatgcgatcgtggtggacccgtccagcaacctgtactaccgctggctgaccgccatcgccctgcctgtcttctataactggtatctgcttatttgcagggcctgtttcgatgagctgcagtccgagtacctgatgctgtggctggtcctggactactcggcagatgtcctgtatgtcttggatgtgcttgtacgagctcggacaggttttcttgagcaaggcttaatggtcagtgataccaacaggctgtggcagcattacaagacgaccacgcagttcaagctggatgtgttgtccctggtccccaccgacctggcttacttaaaggtgggcacaaactacccagaagtgaggttcaaccgcctactgaagttttcccggctctttgaattctttgaccgcacagagacaaggaccaactaccccaatatgttcaggattgggaacttggtcttgtacattctcatcatcatccactggaatgcctgcatctactttgccatttccaagttcattggttttgggacagactcctgggtctacccaaacatctcaatcccagagcatgggcgcctctccaggaagtacatttacagtctctactggtccaccttgacccttaccaccattggtgagaccccaccccccgtgaaagatgaggagtatctctttgtggtcgtagacttcttggtgggtgttctgatttttgccaccattgtgggcaatgtgggctccatgatctcgaatatgaatgcctcacgggcagagttccaggccaagattgattccatcaagcagtacatgcagttccgcaaggtcaccaaggacttggagacgcgggttatccggtggtttgactacctgtgggccaacaagaagacggtggatgagaaggaggtgctcaagagcctcccagacaagctgaaggctgagatcgccatcaacgtgcacctggacacgctgaagaaggttcgcatcttccaggactgtgaggcagggctgctggtggagctggtgctgaagctgcgacccactgtgttcagccctggggattatatctgcaagaagggagatattgggaaggagatgtacatcatcaacgagggcaagctggccgtggtggctgatgatggggtcacccagttcgtggtcctcagcgatggcagctacttcggggagatcagcattctgaacatcaaggggagcaagtcggggaaccgcaggacggccaacatccgcagcattggctactcagacctgttctgcctctcaaaggacgatctcatggaggccctcaccgagtaccccgaagccaagaaggccctggaggagaaaggacggcagatcctgatgaaagacaacctgatcgatgaggagctggccagggcgggcgcggaccccaaggaccttgaggagaaagtggagcagctggggtcctccctggacaccctgcagaccaggtttgcacgcctcctggctgagtacaacgccacccagatgaagatgaagcagcgtctcagccaactggaaagccaggtgaagggtggtggggacaagcccctggctgatggggaagttcccggggatgctacaaaaacagaggacaaacaacagtga

SEQ ID NO: 14 - protein, 694 aa, Homo sapiens; identical to SEQ ID NO: 10

SEQ ID NO: 15 - DNA, 2085 bp, Homo sapiens
atggccaagatcaacacccaatactcccacccctccaggacccacctcaaggtaaagacctcagaccgagatctcaatcgcgctgaaaatggcctcagcagagcccactcgtcaagtgaggagacatcgtcagtgctgcagccggggatcgccatggagaccagaggactggctgactccgggcagggctccttcaccggccaggggatcgccaggctgtcgcgcctcatcttcttgctgcgcaggtgggctgccaggcatgtgcaccaccaggaccagggaccggactcttttcctgatcgtttccgtggagccgagcttaaggaggtgtccagccaagaaagcaatgcccaggcaaatgtgggcagccaggagccagcagacagagggagaagcgcctggcccctggccaaatgcaacactaacaccagcaacaacacggaggaggagaagaagacgaaaaagaaggatgcgatcgtggtggacccgtccagcaacctgtactaccgctggctgaccgccatcgccctgcctgtcttctataactggtatctgcttatttgcagggcctgtttcgatgagctgcagtccgagtacctgatgctgtggctggtcctggactactcggcagatgtcctgtatgtcttggatgtgcttgtacgagctcggacaggttttctcgagcaaggcttaatggtcagtgataccaacaggctgtggcagcattacaagacgaccacgcagttcaagctggatgtgttgtccctggtccccaccgacctggcttacttaaaggtgggcacaaactacccagaagtgaggttcaaccgcctactgaagttttcccggctctttgaattctttgaccgcacagagacaaggaccaactaccccaatatgttcaggattgggaacttggtcttgtacattctcatcatcatccactggaatgcctgcatctactttgccatttccaagttcattggttttgggacagactcctgggtctacccaaacatctcaatcccagagcatgggcgcctctccaggaagtacatttacagtctctactggtccaccttgacccttaccaccattggtgagaccccaccccccgtgaaagatgaggagtatctctttgtggtcgtagacttcttggtgggtgttctgatttttgccaccattgtgggcaatgtgggctccatgatctcgaatatgaatgcctcacgggcagagttccaggccaagattgattccatcaagcagtacatgcagttccgcaaggtcaccaaggacttggagacgcgggttatccggtggtttgactacctgtgggccaacaagaagacggtggatgagaaggaggtgctcaagagcctcccagacaagctgaaggctgagatcgccatcaacgtgcacctggacacgctgaagaaggttcgcatcttccaggactgtgaggcagggctgctggtggagctggtgctgaagctgcgacccactgtgttcagccctggggattatatctgcaagaagggagatattgggaaggagatgtacatcatcaacgagggcaagctggccgtggtggctgatgatggggtcacccagttcgtggtcctcagcgatggcagctacttcggggagatcagcattctgaacatcaaggggagcaagtcggggaaccgcaggacggccaacatccgcagcattggctactcagacctgttctgcctctcaaaggacgatctcatggaggccctcaccgagtaccccgaagccaagaaggccctggaggagaaaggacggcagatcctgatgaaagacaacctgatcgatgaggagctggccagggcgggcgcggaccccaaggaccttgaggagaaagtggagcagctggggtcctccctggacaccctgcagaccaggtttgcacgcctcctggctgagtacaacgccacccagatgaagatgaagcagcgtctcagccaactggaaagccaggtgaagggtggtggggacaagcccctggctgatggggaagttcccggggatgctacaaaaacagaggacaaacaacagtga

SEQ ID NO: 16 - DNA, 2107 bp, Artificial Sequence
  constructed sequence
gcggccgccaccatggctaagattaacacccagtactcacatccatcccgcactcacctcaaagtcaagacctccgatcgggatctgaaccgggctgagaatgggctgtcgcgcgcccactcgtcgtccgaggaaaccagcagcgtgctccagccgggcatcgccatggaaactagggggctggcggactccggacagggatccttcactggacagggtattgcccggctgagcagactgatcttcctgcttcgccgctgggcggccagacacgtgcaccatcaggaccagggacctgatagcttccccgaccgctttaggggagccgagctgaaagaagtgtcaagccaggagtcaaacgcgcaggccaacgtcggcagccaagagcctgcagaccggggacgctcggcatggccgctcgcaaagtgcaacactaacacttccaacaacaccgaagaggaaaagaaaaccaagaagaaggatgcaattgtggtggacccttcctccaacctgtactaccgctggttgaccgccatcgccctcccggtcttttacaattggtatctccttatctgccgggcctgcttcgacgaactgcaatcagagtacctgatgctgtggctggtgctggactatagcgccgatgtgctctacgtcctggatgtgctcgtgcgcgcccggaccggattcttggaacaaggcctgatggtgtccgacacgaatagactgtggcagcactataagaccacaacccagttcaagcttgacgtgctcagccttgtgccgactgacctggcctacctgaaagtcggaactaactacccggaagtcagattcaaccgactcctgaagttcagcaggctgttcgagttctttgaccgcaccgagactcggaccaactaccctaacatgttccggatcggaaatctggtgctctacatactgattatcatccattggaacgcctgtatctatttcgccatttcgaagttcatcggtttcggaaccgattcctgggtgtaccccaacatctcgatccccgaacacggtcgcctgtcccggaagtacatctactccctgtactggtccactctgactctgaccacgatcggggaaacccctccacccgtgaaggacgaagagtacctgttcgtggtggtggacttcctggtcggagtgttgattttcgccaccattgtgggaaacgtgggctccatgatctccaacatgaacgcgtcgagagctgagttccaagccaagatcgactccattaagcagtacatgcagttcagaaaggtcaccaaggacctggaaaccagggtcatccgctggttcgactacctgtgggccaacaaaaagactgtggacgaaaaggaagtgctgaagtcgctgccggataagctgaaggccgaaatcgccattaacgtgcaccttgacaccctgaagaaagtccggatcttccaagactgtgaagccggcctcctggtggagctcgtgctcaagctgcggcccaccgtgttcagcccgggagattacatttgcaagaagggcgatatcggcaaagagatgtacatcatcaacgagggaaagctggccgtggtcgcggacgacggcgtgacccagttcgtggtgctgtccgacggatcctacttcggtgaaatctcaatcctcaacatcaaggggtccaagtccggcaaccggagaactgccaacattcgctccatcggatacagcgacctgttttgcctgtccaaggatgacctgatggaggctctgactgagtaccctgaagcgaagaaggctttggaggaaaaggggcggcagattctgatgaaggacaatttgatcgacgaggagctcgcacgggccggcgccgaccccaaggatctcgaagagaaggtcgaacagctgggttcttcgcttgataccctgcaaacccgattcgcgcggctgctcgccgagtacaacgcgacccagatgaagatgaagcagagactgtcacagttggaatcccaagtcaagggcggaggcgacaagccgctggcggacggggaagtgcccggggacgccaccaagactgaggacaagcagcagtgatcatagatct

SEQ ID NO: 17 - DNA, 2272 bp, Artificial Sequence
  constructed sequence
gcggccgccaccatggctaagattaacacccagtactcacatccatcccgcactcacctcaaagtcaagacctccgatcgggatctgaaccgggctgagaatgggctgtcgcgcgcccactcgtcgtccgaggaaaccagcagcgtgctccagccgggcatcgccatggaaactagggggctggcggactccggacagggatccttcactggacagggtattgcccggttcgggcggattcagaagaagtcccagccggagaaggtcgtgcgggctgccagcaggggcaggccactcattggttggacacagtggtgcgctgaggatggtggagatgaatcggaaatggcactggccggctctcccggatgcagctcgggcccccaagggagactgagcagactgatcttcctgcttcgccgctgggcggccagacacgtgcaccatcaggaccagggacctgatagcttccccgaccgctttaggggagccgagctgaaagaagtgtcaagccaggagtcaaacgcgcaggccaacgtcggcagccaagagcctgcagaccggggacgctcggcatggccgctcgcaaagtgcaacactaacacttccaacaacaccgaagaggaaaagaaaaccaagaagaaggatgcaattgtggtggacccttcctccaacctgtactaccgctggttgaccgccatcgccctcccggtcttttacaattggtatctccttatctgccgggcctgcttcgacgaactgcaatcagagtacctgatgctgtggctggtgctggactatagcgccgatgtgctctacgtcctggatgtgctcgtgcgcgcccggaccggattcttggaacaaggcctgatggtgtccgacacgaatagactgtggcagcactataagaccacaacccagttcaagcttgacgtgctcagccttgtgccgactgacctggcctacctgaaagtcggaactaactacccggaagtcagattcaaccgactcctgaagttcagcaggctgttcgagttctttgaccgcaccgagactcggaccaactaccctaacatgttccggatcggaaatctggtgctctacatactgattatcatccattggaacgcctgtatctatttcgccatttcgaagttcatcggtttcggaaccgattcctgggtgtaccccaacatctcgatccccgaacacggtcgcctgtcccggaagtacatctactccctgtactggtccactctgactctgaccacgatcggggaaacccctccacccgtgaaggacgaagagtacctgttcgtggtggtggacttcctggtcggagtgttgattttcgccaccattgtgggaaacgtgggctccatgatctccaacatgaacgcgtcgagagctgagttccaagccaagatcgactccattaagcagtacatgcagttcagaaaggtcaccaaggacctggaaaccagggtcatccgctggttcgactacctgtgggccaacaaaaagactgtggacgaaaaggaagtgctgaagtcgctgccggataagctgaaggccgaaatcgccattaacgtgcaccttgacaccctgaagaaagtccggatcttccaagactgtgaagccggcctcctggtggagctcgtgctcaagctgcggcccaccgtgttcagcccgggagattacatttgcaagaagggcgatatcggcaaagagatgtacatcatcaacgagggaaagctggccgtggtcgcggacgacggcgtgacccagttcgtggtgctgtccgacggatcctacttcggtgaaatctcaatcctcaacatcaaggggtccaagtccggcaaccggagaactgccaacattcgctccatcggatacagcgacctgttttgcctgtccaaggatgacctgatggaggctctgactgagtaccctgaagcgaagaaggctttggaggaaaaggggcggcagattctgatgaaggacaatttgatcgacgaggagctcgcacgggccggcgccgaccccaaggatctcgaagagaaggtcgaacagctgggttcttcgcttgataccctgcaaacccgattcgcgcggctgctcgccgagtacaacgcgacccagatgaagatgaagcagagactgtcacagttggaatcccaagtcaagggcggaggcgacaagccgctggcggacggggaagtgcccggggacgccaccaagactgaggacaagcagcagtgatcatagatct

SEQ ID NO: 18 - DNA, 2107 bp, Artificial Sequence
  constructed sequence
gcggccgccaccatggccaagatcaacacccaatactcccacccctccaggacccacctcaaggtaaagacctcagaccgggatctcaatcgcgctgaaaatggcctcagcagagcccactcgtcaagtgaggagacatcgtcagtgctgcagccggggatcgccatggagaccagaggactggctgactccgggcagggctccttcaccggccaggggatcgccaggctgtcgcgcctcatcttcttgctgcgcaggtgggctgccaggcatgtgcaccaccaggaccagggaccggactcttttcctgatcgtttccgtggagccgagcttaaggaggtgtccagccaagaaagcaatgcccaggcaaatgtgggcagccaggagccagcagacagagggagaagcgcctggcccctggccaaatgcaacactaacaccagcaacaacacggaggaggagaagaagacgaaaaagaaggatgcgatcgtggtggacccgtccagcaacctgtactaccgctggctgaccgccatcgccctgcctgtcttctataactggtatctgcttatttgcagggcctgtttcgatgagctgcagtccgagtacctgatgctgtggctggtcctggactactcggcagatgtcctgtatgtcttggatgtgcttgtacgagctcggacaggttttcttgagcaaggcttaatggtcagtgataccaacaggctgtggcagcattacaagacgaccacgcagttcaagctggatgtgttgtccctggtccccaccgacctggcttacttaaaggtgggcacaaactacccagaagtgaggttcaaccgcctactgaagttttcccggctctttgaattctttgaccgcacagagacaaggaccaactaccccaatatgttcaggattgggaacttggtcttgtacattctcatcatcatccactggaatgcctgcatctactttgccatttccaagttcattggttttgggacagactcctgggtctacccaaacatctcaatcccagagcatgggcgcctctccaggaagtacatttacagtctctactggtccaccttgacccttaccaccattggtgagaccccaccccccgtgaaagatgaggagtatctctttgtggtcgtagacttcttggtgggtgttctgatttttgccaccattgtgggcaatgtgggctccatgatctcgaatatgaatgcctcacgggcagagttccaggccaagattgattccatcaagcagtacatgcagttccgcaaggtcaccaaggacttggagacgcgggttatccggtggtttgactacctgtgggccaacaagaagacggtggatgagaaggaggtgctcaagagcctcccagacaagctgaaggctgagatcgccatcaacgtgcacctggacacgctgaagaaggttcgcatcttccaggactgtgaggcagggctgctggtggagctggtgctgaagctgcgacccactgtgttcagccctggggattatatctgcaagaagggagatattgggaaggagatgtacatcatcaacgagggcaagctggccgtggtggctgatgatggggtcacccagttcgtggtcctcagcgatggcagctacttcggggagatcagcattctgaacatcaaggggagcaagtcggggaaccgcaggacggccaacatccgcagcattggctactcagacctgttctgcctctcaaaggacgatctcatggaggccctcaccgagtaccccgaagccaagaaggccctggaggagaaaggacggcagatcctgatgaaagacaacctgatcgatgaggagctggccagggcgggcgcggaccccaaggaccttgaggagaaagtggagcagctggggtcctccctggacaccctgcagaccaggtttgcacgcctcctggctgagtacaacgccacccagatgaagatgaagcagcgtctcagccaactggaaagccaggtgaagggtggtggggacaagcccctggctgatggggaagttcccggggatgctacaaaaacagaggacaaacaacagtgatcatagatct

SEQ ID NO: 19 - DNA, 2430 bp, Homo sapiens
  CDS (1)..(2430)
atgtttaaatcgctgacaaaagtcaacaaggtgaagcctataggagagaacaatgagaatgaacaaagttctcgtcggaatgaagaaggctctcacccaagtaatcagtctcagcaaaccacagcacaggaagaaaacaaaggtgaagagaaatctctcaaaaccaagtcaactccagtcacgtctgaagagccacacaccaacatacaagacaaactctccaagaaaaattcctctggagatctgaccacaaaccctgaccctcaaaatgcagcagaaccaactggaacagtgccagagcagaaggaaatggaccccgggaaagaaggtccaaacagcccacaaaacaaaccgcctgcagctcctgttataaatgagtatgccgatgcccagctacacaacctggtgaaaagaatgcgtcaaagaacagccctctacaagaaaaagttggtagagggagatctctcctcacccgaagccagcccacaaactgcaaagcccacggctgtaccaccagtaaaagaaagcgatgataagccaacagaacattactacaggctgttgtggttcaaagtcaaaaagatgcctttaacagagtacttaaagcgaattaaacttccaaacagcatagattcatacacagatcgactctatctcctgtggctcttgcttgtcactcttgcctataactggaactgctgttttataccactgcgcctcgtcttcccatatcaaaccgcagacaacatacactactggcttattgcggacatcatatgtgatatcatctacctttatgatatgctatttatccagcccagactccagtttgtaagaggaggagacataatagtggattcaaatgagctaaggaaacactacaggacttctacaaaatttcagttggatgtcgcatcaataataccatttgatatttgctacctcttctttgggtttaatccaatgtttagagcaaataggatgttaaagtacacttcattttttgaatttaatcatcacctagagtctataatggacaaagcatatatctacagagttattcgaacaactggatacttgctgtttattctgcacattaatgcctgtgtttattactgggcttcaaactatgaaggaattggcactactagatgggtgtatgatggggaaggaaacgagtatctgagatgttattattgggcagttcgaactttaattaccattggtggccttccagaaccacaaactttatttgaaattgtttttcaactcttgaattttttttctggagtttttgtgttctccagtttaattggtcagatgagagatgtgattggagcagctacagccaatcagaactacttccgcgcctgcatggatgacaccattgcctacatgaacaattactccattcctaaacttgtgcaaaagcgagttcggacttggtatgaatatacatgggactctcaaagaatgctagatgagtctgatttgcttaagaccctaccaactacggtccagttagccctcgccattgatgtgaacttcagcatcatcagcaaagtcgacttgttcaagggttgtgatacacagatgatttatgacatgttgctaagattgaaatccgttctctatttgcctggtgactttgtctgcaaaaagggagaaattggcaaggaaatgtatatcatcaagcatggagaagtccaagttcttggaggccctgatggtactaaagttctggttactctgaaagctgggtcggtgtttggagaaatcagccttctagcagcaggaggaggaaaccgtcgaactgccaatgtggtggcccacgggtttgccaatcttttaactctagacaaaaagaccctccaagaaattctagtgcattatccagattctgaaaggatcctcatgaagaaagccagagtgcttttaaagcagaaggctaagaccgcagaagcaacccctccaagaaaagatcttgccctcctcttcccaccgaaagaagagacacccaaactgtttaaaactctcctaggaggcacaggaaaagcaagtcttgcaagactactcaaattgaagcgagagcaagcagctcagaagaaagaaaattctgaaggaggagaggaagaaggaaaagaaaatgaagataaacaaaaagaaaatgaagataaacaaaaagaaaatgaagataaaggaaaagaaaatgaagataaagataaaggaagagagccagaagagaagccactggacagacctgaatgtacagcaagtcctattgcagtggaggaagaaccccactcagttagaaggacagttttacccagagggacttctcgtcaatcactcattatcagcatggctccttctgctgagggcggagaagaggttcttactattgaagtcaaagaaaaggctaagcaataa

SEQ ID NO: 20 - protein, 809 aa, Homo sapiens
MFKSLTKVNKVKPIGENNENEQSSRRNEEGSHPSNQSQQTTAQEENKGEEKSLKTKSTPVTSEEPHTNIQDKLSKKNSSGDLTTNPDPQNAAEPTGTVPEQKEMDPGKEGPNSPQNKPPAAPVINEYADAQLHNLVKRMRQRTALYKKKLVEGDLSSPEASPQTAKPTAVPPVKESDDKPTEHYYRLLWFKVKKMPLTEYLKRIKLPNSIDSYTDRLYLLWLLLVTLAYNWNCCFIPLRLVFPYQTADNIHYWLIADIICDIIYLYDMLFIQPRLQFVRGGDIIVDSNELRKHYRTSTKFQLDVASIIPFDICYLFFGFNPMFRANRMLKYTSFFEFNHHLESIMDKAYIYRVIRTTGYLLFILHINACVYYWASNYEGIGTTRWVYDGEGNEYLRCYYWAVRTLITIGGLPEPQTLFEIVFQLLNFFSGVFVFSSLIGQMRDVIGAATANQNYFRACMDDTIAYMNNYSIPKLVQKRVRTWYEYTWDSQRMLDESDLLKTLPTTVQLALAIDVNFSIISKVDLFKGCDTQMIYDMLLRLKSVLYLPGDFVCKKGEIGKEMYIIKHGEVQVLGGPDGTKVLVTLKAGSVFGEISLLAAGGGNRRTANVVAHGFANLLTLDKKTLQEILVHYPDSERILMKKARVLLKQKAKTAEATPPRKDLALLFPPKEETPKLFKTLLGGTGKASLARLLKLKREQAAQKKENSEGGEEEGKENEDKQKENEDKQKENEDKGKENEDKDKGREPEEKPLDRPECTASPIAVEEEPHSVRRTVLPRGTSRQSLIISMAPSAEGGEEVLTIEVKEKAKQ

SEQ ID NO: 21 - DNA, 2430 bp, Artificial Sequence
  constructed sequence
  CDS (1)..(2430)
atgtttaaatcgctgacaaaagtcaacaaggtgaagcctataggagagaacaatgagaatgaacaaagttctcgtcggaatgaagaaggctctcacccaagtaatcagtctcagcaaaccacagcacaggaagaaaacaaaggtgaagagaaatctctcaaaaccaagtcaactccagtcacgtctgaagagccacacaccaacatacaagacaaactctccaagaaaaattcctctggagatctgaccacaaaccctgaccctcaaaatgcagcagaaccaactggaacagtgccagagcagaaggaaatggaccccgggaaagaaggtccaaacagcccacaaaacaaaccgccagcagctcctgttataaatgagtatgccgatgcccagctacacaacctggtgaaaagaatgcgtcaaagaacagccctctacaagaaaaagttggtagagggagatctctcctcacccgaagccagcccacaaactgcaaagcccacggctgtaccaccagtaaaagaaagcgatgataagccaacagaacattactacaggctgttgtggttcaaagtcaaaaagatgcctttaacagagtacttaaagcgaattaaacttccaaacagcatagattcatacacagatcgactctatctcctgtggctcttgcttgtcactcttgcctataactggaactgctgttttataccactgcgcctcgtcttcccatatcaaaccgcagacaacatacactactggcttattgcggacatcatctgtgatatcatctacctttatgatatgctatttatccagcccagactccagtttgtaagaggaggagacataatagtggattcaaatgagctaaggaaacactacaggacttctacaaaatttcagttggatgtcgcatcaataataccatttgatatttgctacctcttctttgggtttaatccaatgtttagagcaaataggatgttaaagtacacttcattttttgaatttaatcatcacctagagtctataatggacaaagcatatatctacagagttattcgaacaactggatacttgctgtttattctgcacattaatgcctgtgtttattactgggcttcaaactatgaaggaattggcactactagatgggtgtatgatggggaaggaaacgagtatctgagatgttattattgggcagttcgaactttaattaccattggtggccttccagaaccacaaactttatttgaaattgtttttcaactcttgaattttttttctggagtttttgtgttctccagtttaattggtcagatgagagatgtgattggagcagctacagccaatcagaactacttccgcgcctgcatggatgacaccattgcctacatgaacaattactccattcctaaacttgtgcaaaagcgagttcggacttggtatgaatatacatgggactctcaaagaatgctagatgagtctgatttgcttaagaccctaccaactacggtccagttagccctcgccattgatgtgaacttcagcatcatcagcaaagttgacttgttcaagggttgtgatacacagatgatttatgacatgttgctaagattgaaatccgttctctatttgcctggtgactttgtctgcaaaaagggagaaattggcaaggaaatgtatatcatcaagcatggagaagtccaagttcttggaggccctgatggtactaaagttctggttactctgaaagctgggtcggtgtttggagaaatcagccttctagcagcaggaggaggaaaccgtcgaactgccaatgtggtggcccacgggtttgccaatcttttaactctagacaaaaagaccctccaagaaattctagtgcattatccagattctgaaagaatcctcatgaagaaagccagagtgcttttaaagcagaaggctaagaccgcagaagcaacccctccaagaaaagatcttgccctcctcttcccaccgaaagaagagacacccaaactgtttaaaactctcctaggaggcacaggaaaagcaagtcttgcaagactactcaaattgaagcgagagcaagcagctcagaagaaagaaaattctgaaggaggagaggaagaaggaaaagaaaatgaagataaacaaaaagaaaatgaagataaacaaaaagaaaatgaagataaaggaaaagaaaatgaagataaagataaaggaagagagccagaagagaagccactggacagacctgaatgtacagcaagtcctattgcagtggaggaagaaccccactcagttagaaggacagttttacccagagggacttctcgtcaatcactcattatcagcatggctccttctgctgagggcggagaagaggttcttactattgaagtcaaagaaaaggctaagcaatga

SEQ ID NO: 22 - protein, 809 aa, Artificial Sequence; identical to SEQ ID NO: 20
  Synthetic Construct

SEQ ID NO: 23 - DNA, 2454 bp, Artificial Sequence
  constructed sequence
  misc_feature (1)..(12): modified end with NotI site and Kozak
  misc_feature (1)..(8): NotI site for subcloning
  CDS (13)..(2448): ORF with silent mutations (stop codon and restriction sites BamHI, PstI, SalI, and NdeI)
  misc_feature (2440)..(2442): modifed stop codon
  misc_feature (2440)..(2445): BclI site to facilitate addition of epitope tag
  misc_feature (2446)..(2448): additional stop codon
  misc_feature (2449)..(2454): PstI site for subcloning
gcggccgccaccatgtttaaatcgctgacaaaagtcaacaaggtgaagcctataggagagaacaatgagaatgaacaaagttctcgtcggaatgaagaaggctctcacccaagtaatcagtctcagcaaaccacagcacaggaagaaaacaaaggtgaagagaaatctctcaaaaccaagtcaactccagtcacgtctgaagagccacacaccaacatacaagacaaactctccaagaaaaattcctctggagatctgaccacaaaccctgaccctcaaaatgcagcagaaccaactggaacagtgccagagcagaaggaaatggaccccgggaaagaaggtccaaacagcccacaaaacaaaccgccagcagctcctgttataaatgagtatgccgatgcccagctacacaacctggtgaaaagaatgcgtcaaagaacagccctctacaagaaaaagttggtagagggagatctctcctcacccgaagccagcccacaaactgcaaagcccacggctgtaccaccagtaaaagaaagcgatgataagccaacagaacattactacaggctgttgtggttcaaagtcaaaaagatgcctttaacagagtacttaaagcgaattaaacttccaaacagcatagattcatacacagatcgactctatctcctgtggctcttgcttgtcactcttgcctataactggaactgctgttttataccactgcgcctcgtcttcccatatcaaaccgcagacaacatacactactggcttattgcggacatcatctgtgatatcatctacctttatgatatgctatttatccagcccagactccagtttgtaagaggaggagacataatagtggattcaaatgagctaaggaaacactacaggacttctacaaaatttcagttggatgtcgcatcaataataccatttgatatttgctacctcttctttgggtttaatccaatgtttagagcaaataggatgttaaagtacacttcattttttgaatttaatcatcacctagagtctataatggacaaagcatatatctacagagttattcgaacaactggatacttgctgtttattctgcacattaatgcctgtgtttattactgggcttcaaactatgaaggaattggcactactagatgggtgtatgatggggaaggaaacgagtatctgagatgttattattgggcagttcgaactttaattaccattggtggccttccagaaccacaaactttatttgaaattgtttttcaactcttgaattttttttctggagtttttgtgttctccagtttaattggtcagatgagagatgtgattggagcagctacagccaatcagaactacttccgcgcctgcatggatgacaccattgcctacatgaacaattactccattcctaaacttgtgcaaaagcgagttcggacttggtatgaatatacatgggactctcaaagaatgctagatgagtctgatttgcttaagaccctaccaactacggtccagttagccctcgccattgatgtgaacttcagcatcatcagcaaagttgacttgttcaagggttgtgatacacagatgatttatgacatgttgctaagattgaaatccgttctctatttgcctggtgactttgtctgcaaaaagggagaaattggcaaggaaatgtatatcatcaagcatggagaagtccaagttcttggaggccctgatggtactaaagttctggttactctgaaagctgggtcggtgtttggagaaatcagccttctagcagcaggaggaggaaaccgtcgaactgccaatgtggtggcccacgggtttgccaatcttttaactctagacaaaaagaccctccaagaaattctagtgcattatccagattctgaaagaatcctcatgaagaaagccagagtgcttttaaagcagaaggctaagaccgcagaagcaacccctccaagaaaagatcttgccctcctcttcccaccgaaagaagagacacccaaactgtttaaaactctcctaggaggcacaggaaaagcaagtcttgcaagactactcaaattgaagcgagagcaagcagctcagaagaaagaaaattctgaaggaggagaggaagaaggaaaagaaaatgaagataaacaaaaagaaaatgaagataaacaaaaagaaaatgaagataaaggaaaagaaaatgaagataaagataaaggaagagagccagaagagaagccactggacagacctgaatgtacagcaagtcctattgcagtggaggaagaaccccactcagttagaaggacagttttacccagagggacttctcgtcaatcactcattatcagcatggctccttctgctgagggcggagaagaggttcttactattgaagtcaaagaaaaggctaagcaatgatcataactgcag

SEQ ID NO: 24 - protein, 809 aa, Artificial Sequence; identical to SEQ ID NO: 20
  Synthetic Construct

SEQ ID NO: 25 - DNA, 11714 bp, Artificial Sequence
  constructed sequence
  misc_feature (1)..(130): 5' ITR
  misc_feature (241)..(544): CMV enhancer
  misc_feature (546)..(823): chicken beta-actin promoter
  misc_feature (824)..(1795): CBA exon 1 and intron
  misc_feature (1859)..(1864): kozak
  misc_feature (1865)..(3826): human codon optimized CHM (REP-1)
  misc_feature (3847)..(4054): bGH poly(A) signal
  misc_feature (4104)..(4233): 3' ITR
ctgcgcgctcgctcgctcactgaggccgcccgggcaaagcccgggcgtcgggcgacctttggtcgcccggcctcagtgagcgagcgagcgcgcagagagggagtggccaactccatcactaggggttccttgtagttaatgattaacccgccatgctacttatctacgtagcaagctagctagttattaatagtaatcaattacggggtcattagttcatagcccatatatggagttccgcgttacataacttacggtaaatggcccgcctggctgaccgcccaacgacccccgcccattgacgtcaataatgacgtatgttcccatagtaacgccaatagggactttccattgacgtcaatgggtggagtatttacggtaaactgcccacttggcagtacatcaagtgtatcatatgccaagtacgccccctattgacgtcaatgacggtaaatggcccgcctggcattatgcccagtacatgaccttatgggactttcctacttggcagtacatctacgtattagtcatcgctattaacatggtcgaggtgagccccacgttctgcttcactctccccatctcccccccctccccacccccaattttgtatttatttattttttaattattttgtgcagcgatgggggcggggggggggggggggcgcgcgccaggcggggcggggcggggcgaggggcggggcggggcgaggcggagaggtgcggcggcagccaatcagagcggcgcgctccgaaagtttccttttatggcgaggcggcggcggcggcggccctataaaaagcgaagcgcgcggcgggcggggagtcgctgcgacgctgccttcgccccgtgccccgctccgccgccgcctcgcgccgcccgccccggctctgactgaccgcgttactcccacaggtgagcgggcgggacggcccttctcctccgggctgtaattagcgcttggtttaatgacggcttgtttcttttctgtggctgcgtgaaagccttgaggggctccgggagggccctttgtgcggggggagcggctcggggggtgcgtgcgtgtgtgtgtgcgtggggagcgccgcgtgcggctccgcgctgcccggcggctgtgagcgctgcgggcgcggcgcggggctttgtgcgctccgcagtgtgcgcgaggggagcgcggccgggggcggtgccccgcggtgcggggggggctgcgaggggaacaaaggctgcgtgcggggtgtgtgcgtgggggggtgagcagggggtgtgggcgcgtcggtcgggctgcaaccccccctgcacccccctccccgagttgctgagcacggcccggcttcgggtgcggggctccgtacggggcgtggcgcggggctcgccgtgccgggcggggggtggcggcaggtgggggtgccgggcggggcggggccgcctcgggccggggagggctcgggggaggggcgcggcggcccccggagcgccggcggctgtcgaggcgcggcgagccgcagccattgccttttatggtaatcgtgcgagagggcgcagggacttcctttgtcccaaatctgtgcggagccgaaatctgggaggcgccgccgcaccccctctagcgggcgcggggcgaagcggtgcggcgccggcaggaaggaaatgggcggggagggccttcgtgcgtcgccgcgccgccgtccccttctccctctccagcctcggggctgtccgcggggggacggctgccttcgggggggacggggcagggcggggttcggcttctggcgtgtgaccggcggctctagacaattgtactaaccttcttctctttcctctcctgacaggttggtgtacactagcggccgccaccatggctgataccctgccctctgaattcgacgtgattgtgattggaaccggactccctgaatcgatcatcgccgcggcctgttcccggtccggtcggcgcgtgctgcacgtcgattcgagaagctactacggagggaattgggcctcattctccttctccggactgctctcctggctgaaggagtatcaggagaactccgacattgtctccgactcacctgtgtggcaggaccagatcctggaaaacgaggaagcaatagccctgagccggaaggacaagaccatccagcacgtggaggtgttctgttatgcctcccaagacctccatgaggacgtggaagaggctggagcgttgcagaagaatcatgccctcgtgacctccgctaactccaccgaggcagccgacagcgccttcctgccgaccgaggatgaatccctgtcaactatgtcgtgcgaaatgctgaccgaacagactccgagctccgaccccgaaaacgccctggaagtgaacggagcggaagtgaccggcgaaaaggagaaccattgcgacgacaagacttgtgtcccatccacttccgcggaggacatgtccgagaatgtgcctatcgccgaggacaccaccgaacagcccaagaagaacagaatcacgtacagccagatcatcaaggaggggcggaggtttaacatcgatctggtgtcgaagctgctgtacagccgcggtctgctgatcgatctgctcattaagtcgaacgtgtcgagatacgccgagttcaagaacatcacaaggattctcgccttccgggaaggaagagtggaacaagtgccgtgctcccgggccgacgtgttcaactcaaagcaacttaccatggtggaaaagcgcatgctgatgaaattcctgaccttctgcatggagtacgaaaagtaccctgatgagtacaagggttacgaagaaattactttctacgagtacctcaagacccagaagctgaccccgaatctgcagtacattgtgatgcactcaatcgcaatgacctccgaaaccgcctcctcgaccatcgacgggctcaaggccaccaagaacttcctgcactgtttggggcgctacggcaacactccgttcctcttcccgctgtacggccagggagagctgcctcagtgtttctgccggatgtgcgccgtgttcggcggaatctactgtctccgccactcggtccagtgcctggtggtggacaaggaatccaggaagtgcaaagccattattgaccagttcggacaacggatcatttccgagcactttcttgtggaggactcatacttcccggagaacatgtgctctcgggtccagtatcgacagatttccagggcggtgctcattactgaccggagcgtcctcaagaccgatagcgaccagcagatctccatcctgaccgtgccggcggaagaacccggcacttttgccgtgcgcgtgatcgagctttgctcatccaccatgacttgcatgaaaggcacttacctggtgcacctgacgtgcacctcatcgaaaaccgctagagaggacctggaatccgtcgtccaaaagctgttcgtgccttacaccgagatggaaattgaaaacgaacaagtggagaagccccgcatcctttgggccctgtactttaacatgcgcgattcctccgatatctcgcggtcctgctataacgacttgccttcgaacgtctacgtctgctccgggccagactgcggtcttggcaacgacaatgccgtgaagcaggcggaaacactgttccaagagatctgccctaacgaggatttttgcccgccccccccaaaccccgaggatatcatcttggacggagacagcctgcagccagaagcatccgagtccagcgccatcccggaggccaacagcgaaaccttcaaggagagcactaacctgggcaacctggaagagtccagcgaatgatcataggatctctgcctcgactgtgccttctagttgccagccatctgttgtttgcccctcccccgtgccttccttgaccctggaaggtgccactcccactgtcctttcctaataaaatgaggaaattgcatcgcattgtctgagtaggtgtcattctattctggggggtggggtggggcaggacagcaagggggaggattgggaagacaatagcaggcatgctggggactcgagttctacgtagataagtagcatggcgggttaatcattaactacaaggaacccctagtgatggagttggccactccctctctgcgcgctcgctcgctcactgaggccgggcgaccaaaggtcgcccgacgcccgggctttgcccgggcggcctcagtgagcgagcgagcgcgcagccttataaggatatggtgcactctcagtacaatctgctctgatgccgcatagttaagccagccccgacacccgccaacacccgctgacgcgccctgacgggcttgtctgctcccggcatccgcttacagacaagctgtgaccgtctccgggagctgcatgtgtcagaggttttcaccgtcatcaccgaaacgcgcgagacgaaagggcctcgtgatacgcctatttttataggttaatgtcatgataataatggtttcttagacgtcaggtggcacttttcggggaaatgtgcgcggaacccctatttgtttatttttctaaatacattcaaatatgtatccgctcatgagacaataaccctgataaatgcttcaataatattgaaaaaggaagagtatgagccatattcaacgggaaacgtcgaggccgcgattaaattccaacatggatgctgatttatatgggtataaatgggctcgcgataatgtcgggcaatcaggtgcgacaatctatcgcttgtatgggaagcccgatgcgccagagttgtttctgaaacatggcaaaggtagcgttgccaatgatgttacagatgagatggtcagactaaactggctgacggaatttatgccacttccgaccatcaagcattttatccgtactcctgatgatgcatggttactcaccactgcgatccccggaaaaacagcgttccaggtattagaagaatatcctgattcaggtgaaaatattgttgatgcgctggcagtgttcctgcgccggttgcactcgattcctgtttgtaattgtccttttaacagcgatcgcgtatttcgcctcgctcaggcgcaatcacgaatgaataacggtttggttgatgcgagtgattttgatgacgagcgtaatggctggcctgttgaacaagtctggaaagaaatgcataaacttttgccattctcaccggattcagtcgtcactcatggtgatttctcacttgataaccttatttttgacgaggggaaattaataggttgtattgatgttggacgagtcggaatcgcagaccgataccaggatcttgccatcctatggaactgcctcggtgagttttctccttcattacagaaacggctttttcaaaaatatggtattgataatcctgatatgaataaattgcagtttcatttgatgctcgatgagtttttctaaactgtcagaccaagtttactcatatatactttagattgatttaaaacttcatttttaatttaaaaggatctaggtgaagatcctttttgataatctcatgaccaaaatcccttaacgtgagttttcgttccactgagcgtcagaccccgtagaaaagatcaaaggatcttcttgagatcctttttttctgcgcgtaatctgctgcttgcaaacaaaaaaaccaccgctaccagcggtggtttgtttgccggatcaagagctaccaactctttttccgaaggtaactggcttcagcagagcgcagataccaaatactgttcttctagtgtagccgtagttaggccaccacttcaagaactctgtagcaccgcctacatacctcgctctgctaatcctgttaccagtggctgctgccagtggcgataagtcgtgtcttaccgggttggactcaagacgatagttaccggataaggcgcagcggtcgggctgaacggggggttcgtgcacacagcccagcttggagcgaacgacctacaccgaactgagatacctacagcgtgagctatgagaaagcgccacgcttcccgaagggagaaaggcggacaggtatccggtaagcggcagggtcggaacaggagagcgcacgagggagcttccagggggaaacgcctggtatctttatagtcctgtcgggtttcgccacctctgacttgagcgtcgatttttgtgatgctcgtcaggggggcggagcctatggaaaaacgccagcaacgcggcctttttacggttcctggccttttgctggccttttgctcacatgttctttcctgcgttatcccctgattctgtggataaccgtattaccgcctttgagtgagctgataccgctcgccgcagccgaacgaccgagcgcagcgagtcagtgagcgaggaagcggaagagcgcccaatacgcaaaccgcctctccccgcgcgttggccgattcattaatgcaggcgcctgttgatttgagttttgggtttagcgtgacaagtttgcgagggtgatcggagtaatcagtaaatagctctccgcctacaatgacgtcataaccatgatttctggttttctgacgtccgttatcagttccctccgaccacgccagcatatcgaggaacgccttacgttgattattgatttctaccatcttctactccggcttttttagcagcgaagcgtttgataagcgaaccaatcgagtcagtaccgatgtagccgataaacacgctcgttatataagcgagattgctacttagtccggcgaagtcgagaaggtcacgaatgaaccaggcgataatggcgcacatcgttgcgtcgattactgtttttgtaaacgcaccgccattatatctgccgcgaaggtacgccattgcaaacgcaaggattgccccgatgccttgttcctttgccgcgagaatggcggccaacaggtcatgtttttctggcatcttcatgtcttacccccaataaggggatttgctctatttaattaggaataaggtcgattactgatagaacaaatccaggctactgtgtttagtaatcagatttgttcgtgaccgatatgcacgggcaaaacggcaggaggttgttagcgcgacctcctgccacccgctttcacgaaggtcatgtgtaaaaggccgcagcgtaactattactaatgaattcaggacagacagtggctacggctcagtttgggttgtgctgttgctgggcggcgatgacgcctgtacgcatttggtgatccggttctgcttccggtattcgcttaattcagcacaacggaaagagcactggctaaccaggctcgccgactcttcacgattatcgactcaatgctcttacctgttgtgcagatataaaaaatcccgaaaccgttatgcaggctctaactattacctgcgaactgtttcgggattgcattttgcagacctctctgcctgcgatggttggagttccagacgatacgtcgaagtgaccaactaggcggaatcggtagtaagcgccgcctcttttcatctcactaccacaacgagcgaattaacccatcgttgagtcaaatttacccaattttattcaataagtcaatatcatgccgttaatatgttgccatccgtggcaatcatgctgctaacgtgtgaccgcattcaaaatgttgtctgcgattgactcttctttgtggcattgcaccaccagagcgtcatacagcggcttaacagtgcgtgaccaggtgggttgggtaaggtttgggattagcatcgtcacagcgcgatatgctgcgcttgctggcatccttgaatagccgacgcctttgcatcttccgcactctttctcgacaactctcccccacagctctgttttggcaatatcaaccgcacggcctgtaccatggcaatctctgcatcttgcccccggcgtcgcggcactacggcaataatccgcataagcgaatgttgcgagcacttgcagtacctttgccttagtatttccttcaagctttgccacaccacggtatttccccgataccttgtgtgcaaattgcatcagatagttgatagccttttgtttgtcgttctggctgagttcgtgcttaccgcagaatgcagccataccgaatccggcttgtgattgcgccatccccatagcagccatcacatcagtaccggaaagagagtcagaagccgtggcccgtggtgagtcgctcatcatcgggctttttggcgaatgaaatttagctacgctttcgagtctcatgcgccttctccctgtacctgaatcaatgttaggtttccgcagaacactgcgccggtatcgatatacatttggttggcaaacttgagtggtttcactgctggcgtatgaccaaagatgaacgtgtccgcgcctttgatttctttcacgatcccgttttgtgagttgctgattcgttcgcggttccagattacctgctgatgatcaactggctttccaaactcgtattcgtcaaagggataatcggcgtggcagataacatattttttatctttgctcaccagttcgatgattaacggaagttcatctgctttatgggcaagagctttagccagaatttctttgtcgtaatcgagattaaagaaccagccaccgccattaagcagccagtgattaacgtttccacgctctgataagccatcaatcatcatttgctcatggtttccacgtacagctctgaaccaggggaatgtgattaattccaggcattcaacgttctctgcaccacgatcaaccaaatcgcccaccgagataagcaggtcttttttgttgtcgaatccaatcgtatccagtttgttcatcaggttcgtgtagcatccgtgcagatcgccaactacccaaatatttcggtatttgctgccatcaattttttcgtaatagcgcatctctttcactccatccgcgatgaaccatgagaacgtcgttgacgatggcgtgcattttcccgtctttatcatcaacgtattttctgaccgtaccgcgactacatttcagtctgcgtgctacttctgtctgatttccgtatgcttcaacgagcatgtctggaatggtttttactgagaacgtcatgcggcctcacttctgctatttcgcaggtctttgagtttctgttggtactctgccttgatcgccttgcactcttcgatagtccagcgatggcggttatggtttgattcgatttcgtctactgcttcctgcccgatgcggctaatcagttcgacgcgatacggaacgagatttccgcttttgtgctggttgcacaccacgcattgcttgtgaatattgcgttcattaaatcggagttgaggtgccgcagcagttgtccggtaatgtccggcatcccactgagcagacgtgagcgttccgcacgagatacatggtaagtcgcggtctctttctctgatgaaggcgtttacggcttgttgggcttgtttaatccagtaactgcggggctttaaggcgagttttcgaatcttaagtttatctttctgtttctgctcctctcgtcgtcgtttcttctctgctgctttttccgctttttcgcgttctttacttcgtcgttcgagtgctatcttggttccacactctggagagcaccaccactgattagcgaatgcagggtgaaaccattcccggcattcatcgtttttacatcgtcttcgcgctggtttagccatcatcttcttcctcgtgcatcgagctattcggatcgctcatcagttctgcgcagcagtgctcacacacgtgaacttccagcacatgcagcttctgaccgcagttagcgcacgttaaagctcgctcgacgctttcttgttcgtaacttcgattttggtcaatcaccttgttttcctcgcacgacgtcttagccaccggatatcccacaggtgagccgtgtagttgaaggtttttacgtcagattcttttgggattggcttgggtttatttctggtgcgtttcgttggaaggtatttgcagttttcgcagattatgtcggtgatacttcgtcgctgtctcgccacacgtcctccttttcctgcggtagtggtaacacccctgttggtgttctttcacaccggagacaccatcgattccagtaaggttgatttggtcggaagcggttatcttctttgcattcaccgcaccgataacatcgcatcatgcagcttccctcccgaagtcgaaatcaagctgccctccaaatatttcgcatgactcagaacaagagccggtatcgaatcttttagctcgtaccatgtcctgatacagggcttgataatcattttctgaatacattttcgcgataccgtccagcgacattcttcctcggtacataatctcctttggcgtttcccgatgtccgtcacgcacatgggatcccgtgatgacctcattaaaaacacgctgcaatccctcctcatctttgcaggcaagtccgattttttgcgttgattttttaatgcagaatatgcagttaccgagatgttccggtatttgcaaatcgaatggttgttgcttccaccatgcgaggatatcttccttctcaaagtctgacagttcagcaagatatctgattccaggctttggctttagccgcttcggttcatcagctctgatgccaatccacgtggtgtaattccctcgcccgaaatggtcatcacagtatttggtgaagggaacgagttttaatctgtcagtgcagaacgcgccgccgacgtatggagtgccatatttctttaccatatcgataaatggcttcagaacaggcattcgcgtctgaatatcctttggttcccataccgtataaccatttggctgtccaagctccgggttgatatcaacctgcaatacggtgagcggtatatcccagaacttcacaacttccctgacaaaccgatatgtcattggatgttcacaacctgtatccatgaaaacgtaatgcacgtctttacctgcccgtcgcttttgctccattagccagagcaaatatgctgacgtcctgccaccggagaaactaacgacatttatcatgcagccctgtctccccatctcgctttccactccagagccagtctcgcttcgtctgaccacttaacgccacgctctgtaccgaatgcctgtataagctctaatagctccgcaaattcgcctacacgcatcctgctggttgactggcctattaccacaaagccattcccggcaaggttaggaacaacatcctgctgctttaatgctgcggtaaacacacacttccagctttctgcatccagccagcgaccatgccattcaacctgacgagagacgtcacctaagcaggcccatagcttcctgttttggtctaagctgcggttgcgttcctgaatggttactacgattggtttggttgggtctggaaggatttgctgtactgcgtgaatagcgttttgctgatgtgctggagatcgaatttcaaaggttagttttttcatgacttccctctcccccaaataaaaaggctggcacgacaggtttcccgactggaaagcgggcagtgagcgcaacgcaattaatgtgagttagctcactcattaggcaccccaggctttacactttatgcttccggctcgtatgttgtgtggaattgtgagcggataacaatttcacacaggaaacagctatgaccatgattacgccaagctgtcgactctagaggatcccctaataagg

SEQ ID NO: 26 - DNA, 6647 bp, Artificial Sequence
  constructed sequence
  misc_feature (1)..(130): 5' ITR
  misc_feature (241)..(544): CMV enhancer
  misc_feature (546)..(823): chicken beta-actin promoter
  misc_feature (824)..(1795): CBA exon 1 and intron
  misc_feature (1859)..(1864): Kozak
  misc_feature (1865)..(3826): human codon optimized CHM (REM-1)
  misc_feature (3847)..(4054): bGH poly(A) signal
  misc_feature (4104)..(4233): 3' ITR
ctgcgcgctcgctcgctcactgaggccgcccgggcaaagcccgggcgtcgggcgacctttggtcgcccggcctcagtgagcgagcgagcgcgcagagagggagtggccaactccatcactaggggttccttgtagttaatgattaacccgccatgctacttatctacgtagcaagctagctagttattaatagtaatcaattacggggtcattagttcatagcccatatatggagttccgcgttacataacttacggtaaatggcccgcctggctgaccgcccaacgacccccgcccattgacgtcaataatgacgtatgttcccatagtaacgccaatagggactttccattgacgtcaatgggtggagtatttacggtaaactgcccacttggcagtacatcaagtgtatcatatgccaagtacgccccctattgacgtcaatgacggtaaatggcccgcctggcattatgcccagtacatgaccttatgggactttcctacttggcagtacatctacgtattagtcatcgctattaacatggtcgaggtgagccccacgttctgcttcactctccccatctcccccccctccccacccccaattttgtatttatttattttttaattattttgtgcagcgatgggggcggggggggggggggggcgcgcgccaggcggggcggggcggggcgaggggcggggcggggcgaggcggagaggtgcggcggcagccaatcagagcggcgcgctccgaaagtttccttttatggcgaggcggcggcggcggcggccctataaaaagcgaagcgcgcggcgggcggggagtcgctgcgacgctgccttcgccccgtgccccgctccgccgccgcctcgcgccgcccgccccggctctgactgaccgcgttactcccacaggtgagcgggcgggacggcccttctcctccgggctgtaattagcgcttggtttaatgacggcttgtttcttttctgtggctgcgtgaaagccttgaggggctccgggagggccctttgtgcggggggagcggctcggggggtgcgtgcgtgtgtgtgtgcgtggggagcgccgcgtgcggctccgcgctgcccggcggctgtgagcgctgcgggcgcggcgcggggctttgtgcgctccgcagtgtgcgcgaggggagcgcggccgggggcggtgccccgcggtgcggggggggctgcgaggggaacaaaggctgcgtgcggggtgtgtgcgtgggggggtgagcagggggtgtgggcgcgtcggtcgggctgcaaccccccctgcacccccctccccgagttgctgagcacggcccggcttcgggtgcggggctccgtacggggcgtggcgcggggctcgccgtgccgggcggggggtggcggcaggtgggggtgccgggcggggcggggccgcctcgggccggggagggctcgggggaggggcgcggcggcccccggagcgccggcggctgtcgaggcgcggcgagccgcagccattgccttttatggtaatcgtgcgagagggcgcagggacttcctttgtcccaaatctgtgcggagccgaaatctgggaggcgccgccgcaccccctctagcgggcgcggggcgaagcggtgcggcgccggcaggaaggaaatgggcggggagggccttcgtgcgtcgccgcgccgccgtccccttctccctctccagcctcggggctgtccgcggggggacggctgccttcgggggggacggggcagggcggggttcggcttctggcgtgtgaccggcggctctagacaattgtactaaccttcttctctttcctctcctgacaggttggtgtacactagcggccgccaccatggctgataccctgccctctgaattcgacgtgattgtgattggaaccggactccctgaatcgatcatcgccgcggcctgttcccggtccggtcggcgcgtgctgcacgtcgattcgagaagctactacggagggaattgggcctcattctccttctccggactgctctcctggctgaaggagtatcaggagaactccgacattgtctccgactcacctgtgtggcaggaccagatcctggaaaacgaggaagcaatagccctgagccggaaggacaagaccatccagcacgtggaggtgttctgttatgcctcccaagacctccatgaggacgtggaagaggctggagcgttgcagaagaatcatgccctcgtgacctccgctaactccaccgaggcagccgacagcgccttcctgccgaccgaggatgaatccctgtcaactatgtcgtgcgaaatgctgaccgaacagactccgagctccgaccccgaaaacgccctggaagtgaacggagcggaagtgaccggcgaaaaggagaaccattgcgacgacaagacttgtgtcccatccacttccgcggaggacatgtccgagaatgtgcctatcgccgaggacaccaccgaacagcccaagaagaacagaatcacgtacagccagatcatcaaggaggggcggaggtttaacatcgatctggtgtcgaagctgctgtacagccgcggtctgctgatcgatctgctcattaagtcgaacgtgtcgagatacgccgagttcaagaacatcacaaggattctcgccttccgggaaggaagagtggaacaagtgccgtgctcccgggccgacgtgttcaactcaaagcaacttaccatggtggaaaagcgcatgctgatgaaattcctgaccttctgcatggagtacgaaaagtaccctgatgagtacaagggttacgaagaaattactttctacgagtacctcaagacccagaagctgaccccgaatctgcagtacattgtgatgcactcaatcgcaatgacctccgaaaccgcctcctcgaccatcgacgggctcaaggccaccaagaacttcctgcactgtttggggcgctacggcaacactccgttcctcttcccgctgtacggccagggagagctgcctcagtgtttctgccggatgtgcgccgtgttcggcggaatctactgtctccgccactcggtccagtgcctggtggtggacaaggaatccaggaagtgcaaagccattattgaccagttcggacaacggatcatttccgagcactttcttgtggaggactcatacttcccggagaacatgtgctctcgggtccagtatcgacagatttccagggcggtgctcattactgaccggagcgtcctcaagaccgatagcgaccagcagatctccatcctgaccgtgccggcggaagaacccggcacttttgccgtgcgcgtgatcgagctttgctcatccaccatgacttgcatgaaaggcacttacctggtgcacctgacgtgcacctcatcgaaaaccgctagagaggacctggaatccgtcgtccaaaagctgttcgtgccttacaccgagatggaaattgaaaacgaacaagtggagaagccccgcatcctttgggccctgtactttaacatgcgcgattcctccgatatctcgcggtcctgctataacgacttgccttcgaacgtctacgtctgctccgggccagactgcggtcttggcaacgacaatgccgtgaagcaggcggaaacactgttccaagagatctgccctaacgaggatttttgcccgccccccccaaaccccgaggatatcatcttggacggagacagcctgcagccagaagcatccgagtccagcgccatcccggaggccaacagcgaaaccttcaaggagagcactaacctgggcaacctggaagagtccagcgaatgatcataggatctctgcctcgactgtgccttctagttgccagccatctgttgtttgcccctcccccgtgccttccttgaccctggaaggtgccactcccactgtcctttcctaataaaatgaggaaattgcatcgcattgtctgagtaggtgtcattctattctggggggtggggtggggcaggacagcaagggggaggattgggaagacaatagcaggcatgctggggactcgagttctacgtagataagtagcatggcgggttaatcattaactacaaggaacccctagtgatggagttggccactccctctctgcgcgctcgctcgctcactgaggccgggcgaccaaaggtcgcccgacgcccgggctttgcccgggcggcctcagtgagcgagcgagcgcgcagccttataaggatatggtgcactctcagtacaatctgctctgatgccgcatagttaagccagccccgacacccgccaacacccgctgacgcgccctgacgggcttgtctgctcccggcatccgcttacagacaagctgtgaccgtctccgggagctgcatgtgtcagaggttttcaccgtcatcaccgaaacgcgcgagacgaaagggcctcgtgatacgcctatttttataggttaatgtcatgataataatggtttcttagacgtcaggtggcacttttcggggaaatgtgcgcggaacccctatttgtttatttttctaaatacattcaaatatgtatccgctcatgagacaataaccctgataaatgcttcaataatattgaaaaaggaagagtatgagccatattcaacgggaaacgtcgaggccgcgattaaattccaacatggatgctgatttatatgggtataaatgggctcgcgataatgtcgggcaatcaggtgcgacaatctatcgcttgtatgggaagcccgatgcgccagagttgtttctgaaacatggcaaaggtagcgttgccaatgatgttacagatgagatggtcagactaaactggctgacggaatttatgccacttccgaccatcaagcattttatccgtactcctgatgatgcatggttactcaccactgcgatccccggaaaaacagcgttccaggtattagaagaatatcctgattcaggtgaaaatattgttgatgcgctggcagtgttcctgcgccggttgcactcgattcctgtttgtaattgtccttttaacagcgatcgcgtatttcgcctcgctcaggcgcaatcacgaatgaataacggtttggttgatgcgagtgattttgatgacgagcgtaatggctggcctgttgaacaagtctggaaagaaatgcataaacttttgccattctcaccggattcagtcgtcactcatggtgatttctcacttgataaccttatttttgacgaggggaaattaataggttgtattgatgttggacgagtcggaatcgcagaccgataccaggatcttgccatcctatggaactgcctcggtgagttttctccttcattacagaaacggctttttcaaaaatatggtattgataatcctgatatgaataaattgcagtttcatttgatgctcgatgagtttttctaaactgtcagaccaagtttactcatatatactttagattgatttaaaacttcatttttaatttaaaaggatctaggtgaagatcctttttgataatctcatgaccaaaatcccttaacgtgagttttcgttccactgagcgtcagaccccgtagaaaagatcaaaggatcttcttgagatcctttttttctgcgcgtaatctgctgcttgcaaacaaaaaaaccaccgctaccagcggtggtttgtttgccggatcaagagctaccaactctttttccgaaggtaactggcttcagcagagcgcagataccaaatactgttcttctagtgtagccgtagttaggccaccacttcaagaactctgtagcaccgcctacatacctcgctctgctaatcctgttaccagtggctgctgccagtggcgataagtcgtgtcttaccgggttggactcaagacgatagttaccggataaggcgcagcggtcgggctgaacggggggttcgtgcacacagcccagcttggagcgaacgacctacaccgaactgagatacctacagcgtgagctatgagaaagcgccacgcttcccgaagggagaaaggcggacaggtatccggtaagcggcagggtcggaacaggagagcgcacgagggagcttccagggggaaacgcctggtatctttatagtcctgtcgggtttcgccacctctgacttgagcgtcgatttttgtgatgctcgtcaggggggcggagcctatggaaaaacgccagcaacgcggcctttttacggttcctggccttttgctggccttttgctcacatgttctttcctgcgttatcccctgattctgtggataaccgtattaccgcctttgagtgagctgataccgctcgccgcagccgaacgaccgagcgcagcgagtcagtgagcgaggaagcggaagagcgcccaatacgcaaaccgcctctccccgcgcgttggccgattcattaatgcagctggcacgacaggtttcccgactggaaagcgggcagtgagcgcaacgcaattaatgtgagttagctcactcattaggcaccccaggctttacactttatgcttccggctcgtatgttgtgtggaattgtgagcggataacaatttcacacaggaaacagctatgaccatgattacgccaagctgtcgactctagaggatcccctaataagg

SEQ ID NO: 27 - DNA, 11971 bp, Artificial Sequence
  constructed sequence
  misc_feature (1)..(130): 5' ITR
  misc_feature (241)..(544): CMV Enhancer
  misc_feature (546)..(823): chicken beta-actin promoter
  misc_feature (824)..(1795): CBA exon 1 and intron
  misc_feature (1859)..(1864): kozak
  misc_feature (1865)..(3826): human codon optimized CHM (REP-1)
  misc_feature (3847)..(4054): bGH poly(A) signal
  misc_feature (4104)..(4233): 3' ITR
ctgcgcgctcgctcgctcactgaggccgcccgggcaaagcccgggcgtcgggcgacctttggtcgcccggcctcagtgagcgagcgagcgcgcagagagggagtggccaactccatcactaggggttccttgtagttaatgattaacccgccatgctacttatctacgtagcaagctagctagttattaatagtaatcaattacggggtcattagttcatagcccatatatggagttccgcgttacataacttacggtaaatggcccgcctggctgaccgcccaacgacccccgcccattgacgtcaataatgacgtatgttcccatagtaacgccaatagggactttccattgacgtcaatgggtggagtatttacggtaaactgcccacttggcagtacatcaagtgtatcatatgccaagtacgccccctattgacgtcaatgacggtaaatggcccgcctggcattatgcccagtacatgaccttatgggactttcctacttggcagtacatctacgtattagtcatcgctattaacatggtcgaggtgagccccacgttctgcttcactctccccatctcccccccctccccacccccaattttgtatttatttattttttaattattttgtgcagcgatgggggcggggggggggggggggcgcgcgccaggcggggcggggcggggcgaggggcggggcggggcgaggcggagaggtgcggcggcagccaatcagagcggcgcgctccgaaagtttccttttatggcgaggcggcggcggcggcggccctataaaaagcgaagcgcgcggcgggcggggagtcgctgcgacgctgccttcgccccgtgccccgctccgccgccgcctcgcgccgcccgccccggctctgactgaccgcgttactcccacaggtgagcgggcgggacggcccttctcctccgggctgtaattagcgcttggtttaatgacggcttgtttcttttctgtggctgcgtgaaagccttgaggggctccgggagggccctttgtgcggggggagcggctcggggggtgcgtgcgtgtgtgtgtgcgtggggagcgccgcgtgcggctccgcgctgcccggcggctgtgagcgctgcgggcgcggcgcggggctttgtgcgctccgcagtgtgcgcgaggggagcgcggccgggggcggtgccccgcggtgcggggggggctgcgaggggaacaaaggctgcgtgcggggtgtgtgcgtgggggggtgagcagggggtgtgggcgcgtcggtcgggctgcaaccccccctgcacccccctccccgagttgctgagcacggcccggcttcgggtgcggggctccgtacggggcgtggcgcggggctcgccgtgccgggcggggggtggcggcaggtgggggtgccgggcggggcggggccgcctcgggccggggagggctcgggggaggggcgcggcggcccccggagcgccggcggctgtcgaggcgcggcgagccgcagccattgccttttatggtaatcgtgcgagagggcgcagggacttcctttgtcccaaatctgtgcggagccgaaatctgggaggcgccgccgcaccccctctagcgggcgcggggcgaagcggtgcggcgccggcaggaaggaaatgggcggggagggccttcgtgcgtcgccgcgccgccgtccccttctccctctccagcctcggggctgtccgcggggggacggctgccttcgggggggacggggcagggcggggttcggcttctggcgtgtgaccggcggctctagacaattgtactaaccttcttctctttcctctcctgacaggttggtgtacactagcggccgccaccatggctgataccctgccctctgaattcgacgtgattgtgattggaaccggactccctgaatcgatcatcgccgcggcctgttcccggtccggtcggcgcgtgctgcacgtcgattcgagaagctactacggagggaattgggcctcattctccttctccggactgctctcctggctgaaggagtatcaggagaactccgacattgtctccgactcacctgtgtggcaggaccagatcctggaaaacgaggaagcaatagccctgagccggaaggacaagaccatccagcacgtggaggtgttctgttatgcctcccaagacctccatgaggacgtggaagaggctggagcgttgcagaagaatcatgccctcgtgacctccgctaactccaccgaggcagccgacagcgccttcctgccgaccgaggatgaatccctgtcaactatgtcgtgcgaaatgctgaccgaacagactccgagctccgaccccgaaaacgccctggaagtgaacggagcggaagtgaccggcgaaaaggagaaccattgcgacgacaagacttgtgtcccatccacttccgcggaggacatgtccgagaatgtgcctatcgccgaggacaccaccgaacagcccaagaagaacagaatcacgtacagccagatcatcaaggaggggcggaggtttaacatcgatctggtgtcgaagctgctgtacagccgcggtctgctgatcgatctgctcattaagtcgaacgtgtcgagatacgccgagttcaagaacatcacaaggattctcgccttccgggaaggaagagtggaacaagtgccgtgctcccgggccgacgtgttcaactcaaagcaacttaccatggtggaaaagcgcatgctgatgaaattcctgaccttctgcatggagtacgaaaagtaccctgatgagtacaagggttacgaagaaattactttctacgagtacctcaagacccagaagctgaccccgaatctgcagtacattgtgatgcactcaatcgcaatgacctccgaaaccgcctcctcgaccatcgacgggctcaaggccaccaagaacttcctgcactgtttggggcgctacggcaacactccgttcctcttcccgctgtacggccagggagagctgcctcagtgtttctgccggatgtgcgccgtgttcggcggaatctactgtctccgccactcggtccagtgcctggtggtggacaaggaatccaggaagtgcaaagccattattgaccagttcggacaacggatcatttccgagcactttcttgtggaggactcatacttcccggagaacatgtgctctcgggtccagtatcgacagatttccagggcggtgctcattactgaccggagcgtcctcaagaccgatagcgaccagcagatctccatcctgaccgtgccggcggaagaacccggcacttttgccgtgcgcgtgatcgagctttgctcatccaccatgacttgcatgaaaggcacttacctggtgcacctgacgtgcacctcatcgaaaaccgctagagaggacctggaatccgtcgtccaaaagctgttcgtgccttacaccgagatggaaattgaaaacgaacaagtggagaagccccgcatcctttgggccctgtactttaacatgcgcgattcctccgatatctcgcggtcctgctataacgacttgccttcgaacgtctacgtctgctccgggccagactgcggtcttggcaacgacaatgccgtgaagcaggcggaaacactgttccaagagatctgccctaacgaggatttttgcccgccccccccaaaccccgaggatatcatcttggacggagacagcctgcagccagaagcatccgagtccagcgccatcccggaggccaacagcgaaaccttcaaggagagcactaacctgggcaacctggaagagtccagcgaatgatcataggatctctgcctcgactgtgccttctagttgccagccatctgttgtttgcccctcccccgtgccttccttgaccctggaaggtgccactcccactgtcctttcctaataaaatgaggaaattgcatcgcattgtctgagtaggtgtcattctattctggggggtggggtggggcaggacagcaagggggaggattgggaagacaatagcaggcatgctggggactcgagttctacgtagataagtagcatggcgggttaatcattaactacaaggaacccctagtgatggagttggccactccctctctgcgcgctcgctcgctcactgaggccgggcgaccaaaggtcgcccgacgcccgggctttgcccgggcggcctcagtgagcgagcgagcgcgcagccttaattaacctaataaggaaaatgaagggaagttcctatactttctagagaataggaacttctatagggagtcgaataagggcgacacaaaaggtattctaaatgcataataaatactgataacatcttatagtttgtattatattttgtattatcgttgacatgtataattttgatatcaaaaactgattttccctttattattttcgagatttattttcttaattctctttaacaaactagaaatattgtatatacaaaaaatcataaataatagatgaatagtttaattataggtgttcatcaatcgaaaaagcaacgtatcttatttaaagtgcgttgcttttttctcatttataaggttaaataattctcatatatcaagcaaagtgacaggcgcccttaaatattctgacaaatgctctttccctaaactccccccataaaaaaacccgccgaagcgggtttttacgttatttgcggattaacgattactcgttatcagaaccgcccaggatgcctggcagttccctactctcgccgctgcgctcggtcgttcggctgcgggacctcagcgctagcggagtgtatactggcttactatgttggcactgatgagggtgtcagtgaagtgcttcatgtggcaggagaaaaaaggctgcaccggtgcgtcagcagaatatgtgatacaggatatattccgcttcctcgctcactgactcgctacgctcggtcgttcgactgcggcgagcggaaatggcttacgaacggggcggagatttcctggaagatgccaggaagatacttaacagggaagtgagagggccgcggcaaagccgtttttccataggctccgcccccctgacaagcatcacgaaatctgacgctcaaatcagtggtggcgaaacccgacaggactataaagataccaggcgtttccccctggcggctccctcgtgcgctctcctgttcctgcctttcggtttaccggtgtcattccgctgttatggccgcgtttgtctcattccacgcctgacactcagttccgggtaggcagttcgctccaagctggactgtatgcacgaaccccccgttcagtccgaccgctgcgccttatccggtaactatcgtcttgagtccaacccggaaagacatgcaaaagcaccactggcagcagccactggtaattgatttagaggagttagtcttgaagtcatgcgccggttaaggctaaactgaaaggacaagttttggtgactgcgctcctccaagccagttacctcggttcaaagagttggtagctcagagaaccttcgaaaaaccgccctgcaaggcggttttttcgttttcagagcaagagattacgcgcagaccaaaacgatctcaagaagatcatcttattaagctcctttttatttgggggagagggaagtcatgaaaaaactaacctttgaaattcgatctccagcacatcagcaaaacgctattcacgcagtacagcaaatccttccagacccaaccaaaccaatcgtagtaaccattcaggaacgcaaccgcagcttagaccaaaacaggaagctatgggcctgcttaggtgacgtctctcgtcaggttgaatggcatggtcgctggctggatgcagaaagctggaagtgtgtgtttaccgcagcattaaagcagcaggatgttgttcctaaccttgccgggaatggctttgtggtaataggccagtcaaccagcaggatgcgtgtaggcgaatttgcggagctattagagcttatacaggcattcggtacagagcgtggcgttaagtggtcagacgaagcgagactggctctggagtggaaagcgagatggggagacagggctgcatgataaatgtcgttagtttctccggtggcaggacgtcagcatatttgctctggctaatggagcaaaagcgacgggcaggtaaagacgtgcattacgttttcatggatacaggttgtgaacatccaatgacatatcggtttgtcagggaagttgtgaagttctgggatataccgctcaccgtattgcaggttgatatcaacccggagcttggacagccaaatggttatacggtatgggaaccaaaggatattcagacgcgaatgcctgttctgaagccatttatcgatatggtaaagaaatatggcactccatacgtcggcggcgcgttctgcactgacagattaaaactcgttcccttcaccaaatactgtgatgaccatttcgggcgagggaattacaccacgtggattggcatcagagctgatgaaccgaagcggctaaagccaaagcctggaatcagatatcttgctgaactgtcagactttgagaaggaagatatcctcgcatggtggaagcaacaaccattcgatttgcaaataccggaacatctcggtaactgcatattctgcattaaaaaatcaacgcaaaaaatcggacttgcctgcaaagatgaggagggattgcagcgtgtttttaatgaggtcatcacgggatcccatgtgcgtgacggacatcgggaaacgccaaaggagattatgtaccgaggaagaatgtcgctggacggtatcgcgaaaatgtattcagaaaatgattatcaagccctgtatcaggacatggtacgagctaaaagattcgataccggctcttgttctgagtcatgcgaaatatttggagggcagcttgatttcgacttcgggagggaagctgcatgatgcgatgttatcggtgcggtgaatgcaaagaagataaccgcttccgaccaaatcaaccttactggaatcgatggtgtctccggtgtgaaagaacaccaacaggggtgttaccactaccgcaggaaaaggaggacgtgtggcgagacagcgacgaagtatcaccgacataatctgcgaaaactgcaaataccttccaacgaaacgcaccagaaataaacccaagccaatcccaaaagaatctgacgtaaaaaccttcaactacacggctcacctgtgggatatccggtggctaagacgtcgtgcgaggaaaacaaggtgattgaccaaaatcgaagttacgaacaagaaagcgtcgagcgagctttaacgtgcgctaactgcggtcagaagctgcatgtgctggaagttcacgtgtgtgagcactgctgcgcagaactgatgagcgatccgaatagctcgatgcacgaggaagaagatgatggctaaaccagcgcgaagacgatgtaaaaacgatgaatgccgggaatggtttcaccctgcattcgctaatcagtggtggtgctctccagagtgtggaaccaagatagcactcgaacgacgaagtaaagaacgcgaaaaagcggaaaaagcagcagagaagaaacgacgacgagaggagcagaaacagaaagataaacttaagattcgaaaactcgccttaaagccccgcagttactggattaaacaagcccaacaagccgtaaacgccttcatcagagaaagagaccgcgacttaccatgtatctcgtgcggaacgctcacgtctgctcagtgggatgccggacattaccggacaactgctgcggcacctcaactccgatttaatgaacgcaatattcacaagcaatgcgtggtgtgcaaccagcacaaaagcggaaatctcgttccgtatcgcgtcgaactgattagccgcatcgggcaggaagcagtagacgaaatcgaatcaaaccataaccgccatcgctggactatcgaagagtgcaaggcgatcaaggcagagtaccaacagaaactcaaagacctgcgaaatagcagaagtgaggccgcatgacgttctcagtaaaaaccattccagacatgctcgttgaagcatacggaaatcagacagaagtagcacgcagactgaaatgtagtcgcggtacggtcagaaaatacgttgatgataaagacgggaaaatgcacgccatcgtcaacgacgttctcatggttcatcgcggatggagtgaaagagatgcgctattacgaaaaaattgatggcagcaaataccgaaatatttgggtagttggcgatctgcacggatgctacacgaacctgatgaacaaactggatacgattggattcgacaacaaaaaagacctgcttatctcggtgggcgatttggttgatcgtggtgcagagaacgttgaatgcctggaattaatcacattcccctggttcagagctgtacgtggaaaccatgagcaaatgatgattgatggcttatcagagcgtggaaacgttaatcactggctgcttaatggcggtggctggttctttaatctcgattacgacaaagaaattctggctaaagctcttgcccataaagcagatgaacttccgttaatcatcgaactggtgagcaaagataaaaaatatgttatctgccacgccgattatccctttgacgaatacgagtttggaaagccagttgatcatcagcaggtaatctggaaccgcgaacgaatcagcaactcacaaaacgggatcgtgaaagaaatcaaaggcgcggacacgttcatctttggtcatacgccagcagtgaaaccactcaagtttgccaaccaaatgtatatcgataccggcgcagtgttctgcggaaacctaacattgattcaggtacagggagaaggcgcatgagactcgaaagcgtagctaaatttcattcgccaaaaagcccgatgatgagcgactcaccacgggccacggcttctgactctctttccggtactgatgtgatggctgctatggggatggcgcaatcacaagccggattcggtatggctgcattctgcggtaagcacgaactcagccagaacgacaaacaaaaggctatcaactatctgatgcaatttgcacacaaggtatcggggaaataccgtggtgtggcaaagcttgaaggaaatactaaggcaaaggtactgcaagtgctcgcaacattcgcttatgcggattattgccgtagtgccgcgacgccgggggcaagatgcagagattgccatggtacaggccgtgcggttgatattgccaaaacagagctgtgggggagagttgtcgagaaagagtgcggaagatgcaaaggcgtcggctattcaaggatgccagcaagcgcagcatatcgcgctgtgacgatgctaatcccaaaccttacccaacccacctggtcacgcactgttaagccgctgtatgacgctctggtggtgcaatgccacaaagaagagtcaatcgcagacaacattttgaatgcggtcacacgttagcagcatgattgccacggatggcaacatattaacggcatgatattgacttattgaataaaattgggtaaatttgactcaacgatgggttaattcgctcgttgtggtagtgagatgaaaagaggcggcgcttactaccgattccgcctagttggtcacttcgacgtatcgtctggaactccaaccatcgcaggcagagaggtctgcaaaatgcaatcccgaaacagttcgcaggtaatagttagagcctgcataacggtttcgggattttttatatctgcacaacaggtaagagcattgagtcgataatcgtgaagagtcggcgagcctggttagccagtgctctttccgttgtgctgaattaagcgaataccggaagcagaaccggatcaccaaatgcgtacaggcgtcatcgccgcccagcaacagcacaacccaaactgagccgtagccactgtctgtcctgaattcattagtaatagttacgctgcggccttttacacatgaccttcgtgaaagcgggtggcaggaggtcgcgctaacaacctcctgccgttttgcccgtgcatatcggtcacgaacaaatctgattactaaacacagtagcctggatttgttctatcagtaatcgaccttattcctaattaaatagagcaaatccccttattgggggtaagacatgaagatgccagaaaaacatgacctgttggccgccattctcgcggcaaaggaacaaggcatcggggcaatccttgcgtttgcaatggcgtaccttcgcggcagatataatggcggtgcgtttacaaaaacagtaatcgacgcaacgatgtgcgccattatcgcctggttcattcgtgaccttctcgacttcgccggactaagtagcaatctcgcttatataacgagcgtgtttatcggctacatcggtactgactcgattggttcgcttatcaaacgcttcgctgctaaaaaagccggagtagaagatggtagaaatcaataatcaacgtaaggcgttcctcgatatgctggcgtggtcggagggaactgataacggacgtcagaaaaccagaaatcatggttatgacgtcattgtaggcggagagctatttactgattactccgatcaccctcgcaaacttgtcacgctaaacccaaaactcaaatcaacaggcgcagcttttagaaaaactcatcgagcatcaaatgaaactgcaatttattcatatcaggattatcaataccatatttttgaaaaagccgtttctgtaatgaaggagaaaactcaccgaggcagttccataggatggcaagatcctggtatcggtctgcgattccgactcgtccaacatcaatacaacctattaatttcccctcgtcaaaaataaggttatcaagtgagaaatcaccatgagtgacgactgaatccggtgagaatggcaaaagtttatgcatttctttccagacttgttcaacaggccagccattacgctcgtcatcaaaatcactcgcatcaaccaaaccgttattcattcgtgattgcgcctgagcgaggcgaaatacgcgatcgctgttaaaaggacaattacaaacaggaatcgagtgcaaccggcgcaggaacactgccagcgcatcaacaatattttcacctgaatcaggatattcttctaatacctggaacgctgtttttccggggatcgcagtggtgagtaaccatgcatcatcaggagtacggataaaatgcttgatggtcggaagtggcataaattccgtcagccagtttagtctgaccatctcatctgtaacatcattggcaacgctacctttgccatgtttcagaaacaactctggcgcatcgggcttcccatacaagcgatagattgtcgcacctgattgcccgacattatcgcgagcccatttatacccatataaatcagcatccatgttggaatttaatcgcggcctcgacgtttcccgttgaatatggctcatattcttcctttttcaatattattgaagcatttatcagggttattgtctcatgagcggatacatatttgaatgtatttagaaaaataaacaaataggggtcagtgttacaaccaattaaccaattctgaacattatcgcgagcccatttatacctgaatatggctcataacaccccttgtttgcctggcggcagtagcgcggtggtcccacctgaccccatgccgaactcagaagtgaaacgccgtagcgccgatggtagtgtggggactccccatgcgagagtagggaactgccaggcatcaaataaaacgaaaggctcagtcgaaagactgggcctttcgcccgggctaattagggggtgtcgcccttattcgactctatagggaagttcctattctctagaaagtataggaacttctgaaggggggtcgatcgacttaattaagg

SEQ ID NO: 28 - DNA, 6900 bp, Artificial Sequence
  constructed sequence
  misc_feature (1)..(130): 5' ITR
  misc_feature (241)..(544): CMV enhancer
  misc_feature (546)..(823): chicken beta actin promoter
  misc_feature (824)..(1795): CBA exon 1 and intron
  misc_feature (1859)..(1864): kozak
  misc_feature (1865)..(3826): human codon optimized CHM (REP-1)
  misc_feature (3847)..(4054): bGH poly(A) signal
  misc_feature (4104)..(4233): 3' ITR
ctgcgcgctcgctcgctcactgaggccgcccgggcaaagcccgggcgtcgggcgacctttggtcgcccggcctcagtgagcgagcgagcgcgcagagagggagtggccaactccatcactaggggttccttgtagttaatgattaacccgccatgctacttatctacgtagcaagctagctagttattaatagtaatcaattacggggtcattagttcatagcccatatatggagttccgcgttacataacttacggtaaatggcccgcctggctgaccgcccaacgacccccgcccattgacgtcaataatgacgtatgttcccatagtaacgccaatagggactttccattgacgtcaatgggtggagtatttacggtaaactgcccacttggcagtacatcaagtgtatcatatgccaagtacgccccctattgacgtcaatgacggtaaatggcccgcctggcattatgcccagtacatgaccttatgggactttcctacttggcagtacatctacgtattagtcatcgctattaacatggtcgaggtgagccccacgttctgcttcactctccccatctcccccccctccccacccccaattttgtatttatttattttttaattattttgtgcagcgatgggggcggggggggggggggggcgcgcgccaggcggggcggggcggggcgaggggcggggcggggcgaggcggagaggtgcggcggcagccaatcagagcggcgcgctccgaaagtttccttttatggcgaggcggcggcggcggcggccctataaaaagcgaagcgcgcggcgggcggggagtcgctgcgacgctgccttcgccccgtgccccgctccgccgccgcctcgcgccgcccgccccggctctgactgaccgcgttactcccacaggtgagcgggcgggacggcccttctcctccgggctgtaattagcgcttggtttaatgacggcttgtttcttttctgtggctgcgtgaaagccttgaggggctccgggagggccctttgtgcggggggagcggctcggggggtgcgtgcgtgtgtgtgtgcgtggggagcgccgcgtgcggctccgcgctgcccggcggctgtgagcgctgcgggcgcggcgcggggctttgtgcgctccgcagtgtgcgcgaggggagcgcggccgggggcggtgccccgcggtgcggggggggctgcgaggggaacaaaggctgcgtgcggggtgtgtgcgtgggggggtgagcagggggtgtgggcgcgtcggtcgggctgcaaccccccctgcacccccctccccgagttgctgagcacggcccggcttcgggtgcggggctccgtacggggcgtggcgcggggctcgccgtgccgggcggggggtggcggcaggtgggggtgccgggcggggcggggccgcctcgggccggggagggctcgggggaggggcgcggcggcccccggagcgccggcggctgtcgaggcgcggcgagccgcagccattgccttttatggtaatcgtgcgagagggcgcagggacttcctttgtcccaaatctgtgcggagccgaaatctgggaggcgccgccgcaccccctctagcgggcgcggggcgaagcggtgcggcgccggcaggaaggaaatgggcggggagggccttcgtgcgtcgccgcgccgccgtccccttctccctctccagcctcggggctgtccgcggggggacggctgccttcgggggggacggggcagggcggggttcggcttctggcgtgtgaccggcggctctagacaattgtactaaccttcttctctttcctctcctgacaggttggtgtacactagcggccgccaccatggctgataccctgccctctgaattcgacgtgattgtgattggaaccggactccctgaatcgatcatcgccgcggcctgttcccggtccggtcggcgcgtgctgcacgtcgattcgagaagctactacggagggaattgggcctcattctccttctccggactgctctcctggctgaaggagtatcaggagaactccgacattgtctccgactcacctgtgtggcaggaccagatcctggaaaacgaggaagcaatagccctgagccggaaggacaagaccatccagcacgtggaggtgttctgttatgcctcccaagacctccatgaggacgtggaagaggctggagcgttgcagaagaatcatgccctcgtgacctccgctaactccaccgaggcagccgacagcgccttcctgccgaccgaggatgaatccctgtcaactatgtcgtgcgaaatgctgaccgaacagactccgagctccgaccccgaaaacgccctggaagtgaacggagcggaagtgaccggcgaaaaggagaaccattgcgacgacaagacttgtgtcccatccacttccgcggaggacatgtccgagaatgtgcctatcgccgaggacaccaccgaacagcccaagaagaacagaatcacgtacagccagatcatcaaggaggggcggaggtttaacatcgatctggtgtcgaagctgctgtacagccgcggtctgctgatcgatctgctcattaagtcgaacgtgtcgagatacgccgagttcaagaacatcacaaggattctcgccttccgggaaggaagagtggaacaagtgccgtgctcccgggccgacgtgttcaactcaaagcaacttaccatggtggaaaagcgcatgctgatgaaattcctgaccttctgcatggagtacgaaaagtaccctgatgagtacaagggttacgaagaaattactttctacgagtacctcaagacccagaagctgaccccgaatctgcagtacattgtgatgcactcaatcgcaatgacctccgaaaccgcctcctcgaccatcgacgggctcaaggccaccaagaacttcctgcactgtttggggcgctacggcaacactccgttcctcttcccgctgtacggccagggagagctgcctcagtgtttctgccggatgtgcgccgtgttcggcggaatctactgtctccgccactcggtccagtgcctggtggtggacaaggaatccaggaagtgcaaagccattattgaccagttcggacaacggatcatttccgagcactttcttgtggaggactcatacttcccggagaacatgtgctctcgggtccagtatcgacagatttccagggcggtgctcattactgaccggagcgtcctcaagaccgatagcgaccagcagatctccatcctgaccgtgccggcggaagaacccggcacttttgccgtgcgcgtgatcgagctttgctcatccaccatgacttgcatgaaaggcacttacctggtgcacctgacgtgcacctcatcgaaaaccgctagagaggacctggaatccgtcgtccaaaagctgttcgtgccttacaccgagatggaaattgaaaacgaacaagtggagaagccccgcatcctttgggccctgtactttaacatgcgcgattcctccgatatctcgcggtcctgctataacgacttgccttcgaacgtctacgtctgctccgggccagactgcggtcttggcaacgacaatgccgtgaagcaggcggaaacactgttccaagagatctgccctaacgaggatttttgcccgccccccccaaaccccgaggatatcatcttggacggagacagcctgcagccagaagcatccgagtccagcgccatcccggaggccaacagcgaaaccttcaaggagagcactaacctgggcaacctggaagagtccagcgaatgatcataggatctctgcctcgactgtgccttctagttgccagccatctgttgtttgcccctcccccgtgccttccttgaccctggaaggtgccactcccactgtcctttcctaataaaatgaggaaattgcatcgcattgtctgagtaggtgtcattctattctggggggtggggtggggcaggacagcaagggggaggattgggaagacaatagcaggcatgctggggactcgagttctacgtagataagtagcatggcgggttaatcattaactacaaggaacccctagtgatggagttggccactccctctctgcgcgctcgctcgctcactgaggccgggcgaccaaaggtcgcccgacgcccgggctttgcccgggcggcctcagtgagcgagcgagcgcgcagccttaattaacctaataaggaaaatgaagggaagttcctatactttctagagaataggaacttctatagggagtcgaataagggcgacacaaaaggtattctaaatgcataataaatactgataacatcttatagtttgtattatattttgtattatcgttgacatgtataattttgatatcaaaaactgattttccctttattattttcgagatttattttcttaattctctttaacaaactagaaatattgtatatacaaaaaatcataaataatagatgaatagtttaattataggtgttcatcaatcgaaaaagcaacgtatcttatttaaagtgcgttgcttttttctcatttataaggttaaataattctcatatatcaagcaaagtgacaggcgcccttaaatattctgacaaatgctctttccctaaactccccccataaaaaaacccgccgaagcgggtttttacgttatttgcggattaacgattactcgttatcagaaccgcccaggatgcctggcagttccctactctcgccgctgcgctcggtcgttcggctgcgggacctcagcgctagcggagtgtatactggcttactatgttggcactgatgagggtgtcagtgaagtgcttcatgtggcaggagaaaaaaggctgcaccggtgcgtcagcagaatatgtgatacaggatatattccgcttcctcgctcactgactcgctacgctcggtcgttcgactgcggcgagcggaaatggcttacgaacggggcggagatttcctggaagatgccaggaagatacttaacagggaagtgagagggccgcggcaaagccgtttttccataggctccgcccccctgacaagcatcacgaaatctgacgctcaaatcagtggtggcgaaacccgacaggactataaagataccaggcgtttccccctggcggctccctcgtgcgctctcctgttcctgcctttcggtttaccggtgtcattccgctgttatggccgcgtttgtctcattccacgcctgacactcagttccgggtaggcagttcgctccaagctggactgtatgcacgaaccccccgttcagtccgaccgctgcgccttatccggtaactatcgtcttgagtccaacccggaaagacatgcaaaagcaccactggcagcagccactggtaattgatttagaggagttagtcttgaagtcatgcgccggttaaggctaaactgaaaggacaagttttggtgactgcgctcctccaagccagttacctcggttcaaagagttggtagctcagagaaccttcgaaaaaccgccctgcaaggcggttttttcgttttcagagcaagagattacgcgcagaccaaaacgatctcaagaagatcatcttattaagcttttagaaaaactcatcgagcatcaaatgaaactgcaatttattcatatcaggattatcaataccatatttttgaaaaagccgtttctgtaatgaaggagaaaactcaccgaggcagttccataggatggcaagatcctggtatcggtctgcgattccgactcgtccaacatcaatacaacctattaatttcccctcgtcaaaaataaggttatcaagtgagaaatcaccatgagtgacgactgaatccggtgagaatggcaaaagtttatgcatttctttccagacttgttcaacaggccagccattacgctcgtcatcaaaatcactcgcatcaaccaaaccgttattcattcgtgattgcgcctgagcgaggcgaaatacgcgatcgctgttaaaaggacaattacaaacaggaatcgagtgcaaccggcgcaggaacactgccagcgcatcaacaatattttcacctgaatcaggatattcttctaatacctggaacgctgtttttccggggatcgcagtggtgagtaaccatgcatcatcaggagtacggataaaatgcttgatggtcggaagtggcataaattccgtcagccagtttagtctgaccatctcatctgtaacatcattggcaacgctacctttgccatgtttcagaaacaactctggcgcatcgggcttcccatacaagcgatagattgtcgcacctgattgcccgacattatcgcgagcccatttatacccatataaatcagcatccatgttggaatttaatcgcggcctcgacgtttcccgttgaatatggctcatattcttcctttttcaatattattgaagcatttatcagggttattgtctcatgagcggatacatatttgaatgtatttagaaaaataaacaaataggggtcagtgttacaaccaattaaccaattctgaacattatcgcgagcccatttatacctgaatatggctcataacaccccttgtttgcctggcggcagtagcgcggtggtcccacctgaccccatgccgaactcagaagtgaaacgccgtagcgccgatggtagtgtggggactccccatgcgagagtagggaactgccaggcatcaaataaaacgaaaggctcagtcgaaagactgggcctttcgcccgggctaattagggggtgtcgcccttattcgactctatagggaagttcctattctctagaaagtataggaacttctgaaggggggtcgatcgacttaattaagg

SEQ ID NO: 29 - DNA, 12074 bp, Artificial Sequence
  constructed sequence
ctgcgcgctcgctcgctcactgaggccgcccgggcaaagcccgggcgtcgggcgacctttggtcgcccggcctcagtgagcgagcgagcgcgcagagagggagtggccaactccatcactaggggttccttgtagttaatgattaacccgccatgctacttatctacgtagcaagctagctagttattaatagtaatcaattacggggtcattagttcatagcccatatatggagttccgcgttacataacttacggtaaatggcccgcctggctgaccgcccaacgacccccgcccattgacgtcaataatgacgtatgttcccatagtaacgccaatagggactttccattgacgtcaatgggtggagtatttacggtaaactgcccacttggcagtacatcaagtgtatcatatgccaagtacgccccctattgacgtcaatgacggtaaatggcccgcctggcattatgcccagtacatgaccttatgggactttcctacttggcagtacatctacgtattagtcatcgctattaacatggtcgaggtgagccccacgttctgcttcactctccccatctcccccccctccccacccccaattttgtatttatttattttttaattattttgtgcagcgatgggggcggggggggggggggggcgcgcgccaggcggggcggggcggggcgaggggcggggcggggcgaggcggagaggtgcggcggcagccaatcagagcggcgcgctccgaaagtttccttttatggcgaggcggcggcggcggcggccctataaaaagcgaagcgcgcggcgggcggggagtcgctgcgacgctgccttcgccccgtgccccgctccgccgccgcctcgcgccgcccgccccggctctgactgaccgcgttactcccacaggtgagcgggcgggacggcccttctcctccgggctgtaattagcgcttggtttaatgacggcttgtttcttttctgtggctgcgtgaaagccttgaggggctccgggagggccctttgtgcggggggagcggctcggggggtgcgtgcgtgtgtgtgtgcgtggggagcgccgcgtgcggctccgcgctgcccggcggctgtgagcgctgcgggcgcggcgcggggctttgtgcgctccgcagtgtgcgcgaggggagcgcggccgggggcggtgccccgcggtgcggggggggctgcgaggggaacaaaggctgcgtgcggggtgtgtgcgtgggggggtgagcagggggtgtgggcgcgtcggtcgggctgcaaccccccctgcacccccctccccgagttgctgagcacggcccggcttcgggtgcggggctccgtacggggcgtggcgcggggctcgccgtgccgggcggggggtggcggcaggtgggggtgccgggcggggcggggccgcctcgggccggggagggctcgggggaggggcgcggcggcccccggagcgccggcggctgtcgaggcgcggcgagccgcagccattgccttttatggtaatcgtgcgagagggcgcagggacttcctttgtcccaaatctgtgcggagccgaaatctgggaggcgccgccgcaccccctctagcgggcgcggggcgaagcggtgcggcgccggcaggaaggaaatgggcggggagggccttcgtgcgtcgccgcgccgccgtccccttctccctctccagcctcggggctgtccgcggggggacggctgccttcgggggggacggggcagggcggggttcggcttctggcgtgtgaccggcggctctagacaattgtactaaccttcttctctttcctctcctgacaggttggtgtacactagcggccgcatggcggatactctcccttcggagtttgatgtgatcgtaatagggacgggtttgcctgaatccatcattgcagctgcatgttcaagaagtggccggagagttctgcatgttgattcaagaagctactatggaggaaactgggccagttttagcttttcaggactattgtcctggctaaaggaataccaggaaaacagtgacattgtaagtgacagtccagtgtggcaagaccagatccttgaaaatgaagaagccattgctcttagcaggaaggacaaaactattcaacatgtggaagtattttgttatgccagtcaggatttgcatgaagatgtcgaagaagctggtgcactgcagaaaaatcatgctcttgtgacatctgcaaactccacagaagctgcagattctgccttcctgcctacggaggatgagtcattaagcactatgagctgtgaaatgctcacagaacaaactccaagcagcgatccagagaatgcgctagaagtaaatggtgctgaagtgacaggggaaaaagaaaaccattgtgatgataaaacttgtgtgccatcaacttcagcagaagacatgagtgaaaatgtgcctatagcagaagataccacagagcaaccaaagaaaaacagaattacttactcacaaattattaaagaaggcaggagatttaatattgatttagtatcaaagctgctgtattctcgaggattactaattgatcttctaatcaaatctaatgttagtcgatatgcagagtttaaaaatattaccaggattcttgcatttcgagaaggacgagtggaacaggttccgtgttccagagcagatgtctttaatagcaaacaacttactatggtagaaaagcgaatgctaatgaaatttcttacattttgtatggaatatgagaaatatcctgatgaatataaaggatatgaagagatcacattttatgaatatttaaagactcaaaaattaacccccaacctccaatatattgtcatgcattcaattgcaatgacatcagagacagccagcagcaccatagatggtctcaaagctaccaaaaactttcttcactgtcttgggcggtatggcaacactccatttttgtttcctttatatggccaaggagaactcccccagtgtttctgcaggatgtgtgctgtgtttggtggaatttattgtcttcgccattcagtacagtgccttgtagtggacaaagaatccagaaaatgtaaagcaattatagatcagtttggtcagagaataatctctgagcatttcctcgtggaggacagttactttcctgagaacatgtgctcacgtgtgcaatacaggcagatctccagggcagtgctgattacagatagatctgtcctaaaaacagattcagatcaacagatttccattttgacagtgccagcagaggaaccaggaacttttgctgttcgggtcattgagttatgttcttcaacgatgacatgcatgaaaggcacctatttggttcatttgacttgcacatcttctaaaacagcaagagaagatttagaatcagttgtgcagaaattgtttgttccatatactgaaatggagatagaaaatgaacaagtagaaaagccaagaattctgtgggctctttacttcaatatgagagattcgtcagacatcagcaggagctgttataatgatttaccatccaacgtttatgtctgctctggcccagattgtggtttaggaaatgataatgcagtcaaacaggctgaaacacttttccaggaaatctgccccaatgaagatttctgtccccctccaccaaatcctgaagacattatccttgatggagacagtttacagccagaggcttcagaatccagtgccataccagaggctaactcggagactttcaaggaaagcacaaaccttggaaacctagaggagtcctctgaataaggatctgcctcgactgtgccttctagttgccagccatctgttgtttgcccctcccccgtgccttccttgaccctggaaggtgccactcccactgtcctttcctaataaaatgaggaaattgcatcgcattgtctgagtaggtgtcattctattctggggggtggggtggggcaggacagcaagggggaggattgggaagacaatagcaggcatgctggggactcgagttctacgtagataagtagcatggcgggttaatcattaactacaaggaacccctagtgatggagttggccactccctctctgcgcgctcgctcgctcactgaggccgggcgaccaaaggtcgcccgacgcccgggctttgcccgggcggcctcagtgagcgagcgagcgcgcagccttaattaacctaaggaaaatgaagtgaagttcctatactttctagagaataggaacttctatagtgagtcgaataagggcgacacaaaatttattctaaatgcataataaatactgataacatcttatagtttgtattatattttgtattatcgttgacatgtataattttgatatcaaaaactgattttccctttattattttcgagatttattttcttaattctctttaacaaactagaaatattgtatatacaaaaaatcataaataatagatgaatagtttaattataggtgttcatcaatcgaaaaagcaacgtatcttatttaaagtgcgttgcttttttctcatttataaggttaaataattctcatatatcaagcaaagtgacaggcgcccttaaatattctgacaaatgctctttccctaaactccccccataaaaaaacccgccgaagcgggtttttacgttatttgcggattaacgattactcgttatcagaaccgcccagggggcccgagcttaacctttttatttgggggagagggaagtcatgaaaaaactaacctttgaaattcgatctccagcacatcagcaaaacgctattcacgcagtacagcaaatccttccagacccaaccaaaccaatcgtagtaaccattcaggaacgcaaccgcagcttagaccaaaacaggaagctatgggcctgcttaggtgacgtctctcgtcaggttgaatggcatggtcgctggctggatgcagaaagctggaagtgtgtgtttaccgcagcattaaagcagcaggatgttgttcctaaccttgccgggaatggctttgtggtaataggccagtcaaccagcaggatgcgtgtaggcgaatttgcggagctattagagcttatacaggcattcggtacagagcgtggcgttaagtggtcagacgaagcgagactggctctggagtggaaagcgagatggggagacagggctgcatgataaatgtcgttagtttctccggtggcaggacgtcagcatatttgctctggctaatggagcaaaagcgacgggcaggtaaagacgtgcattacgttttcatggatacaggttgtgaacatccaatgacatatcggtttgtcagggaagttgtgaagttctgggatataccgctcaccgtattgcaggttgatatcaacccggagcttggacagccaaatggttatacggtatgggaaccaaaggatattcagacgcgaatgcctgttctgaagccatttatcgatatggtaaagaaatatggcactccatacgtcggcggcgcgttctgcactgacagattaaaactcgttcccttcaccaaatactgtgatgaccatttcgggcgagggaattacaccacgtggattggcatcagagctgatgaaccgaagcggctaaagccaaagcctggaatcagatatcttgctgaactgtcagactttgagaaggaagatatcctcgcatggtggaagcaacaaccattcgatttgcaaataccggaacatctcggtaactgcatattctgcattaaaaaatcaacgcaaaaaatcggacttgcctgcaaagatgaggagggattgcagcgtgtttttaatgaggtcatcacgggatcccatgtgcgtgacggacatcgggaaacgccaaaggagattatgtaccgaggaagaatgtcgctggacggtatcgcgaaaatgtattcagaaaatgattatcaagccctgtatcaggacatggtacgagctaaaagattcgataccggctcttgttctgagtcatgcgaaatatttggagggcagcttgatttcgacttcgggagggaagctgcatgatgcgatgttatcggtgcggtgaatgcaaagaagataaccgcttccgaccaaatcaaccttactggaatcgatggtgtctccggtgtgaaagaacaccaacaggggtgttaccactaccgcaggaaaaggaggacgtgtggcgagacagcgacgaagtatcaccgacataatctgcgaaaactgcaaataccttccaacgaaacgcaccagaaataaacccaagccaatcccaaaagaatctgacgtaaaaaccttcaactacacggctcacctgtgggatatccggtggctaagacgtcgtgcgaggaaaacaaggtgattgaccaaaatcgaagttacgaacaagaaagcgtcgagcgagctttaacgtgcgctaactgcggtcagaagctgcatgtgctggaagttcacgtgtgtgagcactgctgcgcagaactgatgagcgatccgaatagctcgatgcacgaggaagaagatgatggctaaaccagcgcgaagacgatgtaaaaacgatgaatgccgggaatggtttcaccctgcattcgctaatcagtggtggtgctctccagagtgtggaaccaagatagcactcgaacgacgaagtaaagaacgcgaaaaagcggaaaaagcagcagagaagaaacgacgacgagaggagcagaaacagaaagataaacttaagattcgaaaactcgccttaaagccccgcagttactggattaaacaagcccaacaagccgtaaacgccttcatcagagaaagagaccgcgacttaccatgtatctcgtgcggaacgctcacgtctgctcagtgggatgccggacattaccggacaactgctgcggcacctcaactccgatttaatgaacgcaatattcacaagcaatgcgtggtgtgcaaccagcacaaaagcggaaatctcgttccgtatcgcgtcgaactgattagccgcatcgggcaggaagcagtagacgaaatcgaatcaaaccataaccgccatcgctggactatcgaagagtgcaaggcgatcaaggcagagtaccaacagaaactcaaagacctgcgaaatagcagaagtgaggccgcatgacgttctcagtaaaaaccattccagacatgctcgttgaagcatacggaaatcagacagaagtagcacgcagactgaaatgtagtcgcggtacggtcagaaaatacgttgatgataaagacgggaaaatgcacgccatcgtcaacgacgttctcatggttcatcgcggatggagtgaaagagatgcgctattacgaaaaaattgatggcagcaaataccgaaatatttgggtagttggcgatctgcacggatgctacacgaacctgatgaacaaactggatacgattggattcgacaacaaaaaagacctgcttatctcggtgggcgatttggttgatcgtggtgcagagaacgttgaatgcctggaattaatcacattcccctggttcagagctgtacgtggaaaccatgagcaaatgatgattgatggcttatcagagcgtggaaacgttaatcactggctgcttaatggcggtggctggttctttaatctcgattacgacaaagaaattctggctaaagctcttgcccataaagcagatgaacttccgttaatcatcgaactggtgagcaaagataaaaaatatgttatctgccacgccgattatccctttgacgaatacgagtttggaaagccagttgatcatcagcaggtaatctggaaccgcgaacgaatcagcaactcacaaaacgggatcgtgaaagaaatcaaaggcgcggacacgttcatctttggtcatacgccagcagtgaaaccactcaagtttgccaaccaaatgtatatcgataccggcgcagtgttctgcggaaacctaacattgattcaggtacagggagaaggcgcatgagactcgaaagcgtagctaaatttcattcgccaaaaagcccgatgatgagcgactcaccacgggccacggcttctgactctctttccggtactgatgtgatggctgctatggggatggcgcaatcacaagccggattcggtatggctgcattctgcggtaagcacgaactcagccagaacgacaaacaaaaggctatcaactatctgatgcaatttgcacacaaggtatcggggaaataccgtggtgtggcaaagcttgaaggaaatactaaggcaaaggtactgcaagtgctcgcaacattcgcttatgcggattattgccgtagtgccgcgacgccgggggcaagatgcagagattgccatggtacaggccgtgcggttgatattgccaaaacagagctgtgggggagagttgtcgagaaagagtgcggaagatgcaaaggcgtcggctattcaaggatgccagcaagcgcagcatatcgcgctgtgacgatgctaatcccaaaccttacccaacccacctggtcacgcactgttaagccgctgtatgacgctctggtggtgcaatgccacaaagaagagtcaatcgcagacaacattttgaatgcggtcacacgttagcagcatgattgccacggatggcaacatattaacggcatgatattgacttattgaataaaattgggtaaatttgactcaacgatgggttaattcgctcgttgtggtagtgagatgaaaagaggcggcgcttactaccgattccgcctagttggtcacttcgacgtatcgtctggaactccaaccatcgcaggcagagaggtctgcaaaatgcaatcccgaaacagttcgcaggtaatagttagagcctgcataacggtttcgggattttttatatctgcacaacaggtaagagcattgagtcgataatcgtgaagagtcggcgagcctggttagccagtgctctttccgttgtgctgaattaagcgaataccggaagcagaaccggatcaccaaatgcgtacaggcgtcatcgccgcccagcaacagcacaacccaaactgagccgtagccactgtctgtcctgaattcattagtaatagttacgctgcggccttttacacatgaccttcgtgaaagcgggtggcaggaggtcgcgctaacaacctcctgccgttttgcccgtgcatatcggtcacgaacaaatctgattactaaacacagtagcctggatttgttctatcagtaatcgaccttattcctaattaaatagagcaaatccccttattgggggtaagacatgaagatgccagaaaaacatgacctgttggccgccattctcgcggcaaaggaacaaggcatcggggcaatccttgcgtttgcaatggcgtaccttcgcggcagatataatggcggtgcgtttacaaaaacagtaatcgacgcaacgatgtgcgccattatcgcctggttcattcgtgaccttctcgacttcgccggactaagtagcaatctcgcttatataacgagcgtgtttatcggctacatcggtactgactcgattggttcgcttatcaaacgcttcgctgctaaaaaagccggagtagaagatggtagaaatcaataatcaacgtaaggcgttcctcgatatgctggcgtggtcggagggaactgataacggacgtcagaaaaccagaaatcatggttatgacgtcattgtaggcggagagctatttactgattactccgatcaccctcgcaaacttgtcacgctaaacccaaaactcaaatcaacaggcgcttaagactggccgtcgttttacaacacagaaagagtttgtagaaacgcaaaaaggccatccgtcaggggccttctgcttagtttgatgcctggcagttccctactctcgccttccgcttcctcgctcactgactcgctgcgctcggtcgttcggctgcggcgagcggtatcagctcactcaaaggcggtaatacggttatccacagaatcaggggataacgcaggaaagaacatgtgagcaaaaggccagcaaaaggccaggaaccgtaaaaaggccgcgttgctggcgtttttccataggctccgcccccctgacgagcatcacaaaaatcgacgctcaagtcagaggtggcgaaacccgacaggactataaagataccaggcgtttccccctggaagctccctcgtgcgctctcctgttccgaccctgccgcttaccggatacctgtccgcctttctcccttcgggaagcgtggcgctttctcatagctcacgctgtaggtatctcagttcggtgtaggtcgttcgctccaagctgggctgtgtgcacgaaccccccgttcagcccgaccgctgcgccttatccggtaactatcgtcttgagtccaacccggtaagacacgacttatcgccactggcagcagccactggtaacaggattagcagagcgaggtatgtaggcggtgctacagagttcttgaagtggtgggctaactacggctacactagaagaacagtatttggtatctgcgctctgctgaagccagttaccttcggaaaaagagttggtagctcttgatccggcaaacaaaccaccgctggtagcggtggtttttttgtttgcaagcagcagattacgcgcagaaaaaaaggatctcaagaagatcctttgatcttttctacggggtctgacgctcagtggaacgacgcgcgcgtaactcacgttaagggattttggtcatgagcttgcgccgtcccgtcaagtcagcgtaatgctctgcttttagaaaaactcatcgagcatcaaatgaaactgcaatttattcatatcaggattatcaataccatatttttgaaaaagccgtttctgtaatgaaggagaaaactcaccgaggcagttccataggatggcaagatcctggtatcggtctgcgattccgactcgtccaacatcaatacaacctattaatttcccctcgtcaaaaataaggttatcaagtgagaaatcaccatgagtgacgactgaatccggtgagaatggcaaaagtttatgcatttctttccagacttgttcaacaggccagccattacgctcgtcatcaaaatcactcgcatcaaccaaaccgttattcattcgtgattgcgcctgagcgaggcgaaatacgcgatcgctgttaaaaggacaattacaaacaggaatcgagtgcaaccggcgcaggaacactgccagcgcatcaacaatattttcacctgaatcaggatattcttctaatacctggaacgctgtttttccggggatcgcagtggtgagtaaccatgcatcatcaggagtacggataaaatgcttgatggtcggaagtggcataaattccgtcagccagtttagtctgaccatctcatctgtaacatcattggcaacgctacctttgccatgtttcagaaacaactctggcgcatcgggcttcccatacaagcgatagattgtcgcacctgattgcccgacattatcgcgagcccatttatacccatataaatcagcatccatgttggaatttaatcgcggcctcgacgtttcccgttgaatatggctcatattcttcctttttcaatattattgaagcatttatcagggttattgtctcatgagcggatacatatttgaatgtatttagaaaaataaacaaataggggtcagtgttacaaccaattaaccaattctgaacattatcgcgagcccatttatacctgaatatggctcataacaccccttgtttgcctggcggcagtagcgcggtggtcccacctgaccccatgccgaactcagaagtgaaacgccgtagcgccgatggtagtgtggggactccccatgcgagagtagggaactgccaggcatcaaataaaacgaaaggctcagtcgaaagactgggcctttcgcccgggctaattagggggtgtcgcccttattcgactctatagtgaagttcctattctctagaaagtataggaacttctgaagtggggtcgacttaattaagg